European Patent Application EP 4 566 623 A2, published June 11, 2025. Title: Caninized antibodies. Applicant: Intervet International BV. Application EP. The sequence listing filed with the application follows.

SEQUENCE LISTING (146 sequences)

SEQ ID NO: 1 - DNA, 690 bp, synthetic construct
  misc_feature 1..690: note = modified canine sequence
  misc_difference 10..12: note = n is a, c, g, or t
  misc_difference 91..93: note = n is a, c, g, or t
  misc_difference 187..195: note = n is a, c, g, or t
  misc_difference 277..279: note = n is a, c, g, or t
  misc_difference 283..285: note = n is a, c, g, or t
  source 1..690: mol_type = other DNA
ctgggcggcnnnagcgtgtttatttttccgccgaaaccgaaagataccctgctgattgcgcgcaccccggaagtgacctgcgtggtggtgnnnctggatccggaagatccggaagtgcagattagctggtttgtggatggcaaacagatgcagaccgcgaaaacccagccgcgcgaagaacagtttnnnnnnnnntatcgcgtggtgagcgtgctgccgattggccatcaggattggctgaaaggcaaacagtttacctgcaaagtgaacaacaaannnctgnnnagcccgattgaacgcaccattagcaaagcgcgcggccaggcgcatcagccgagcgtgtatgtgctgccgccgagccgcgaagaactgagcaaaaacaccgtgagcctgacctgcctgattaaagatttttttccgccggatattgatgtggaatggcagagcaacggccagcaggaaccggaaagcaaatatcgcaccaccccgccgcagctggatgaagatggcagctattttctgtatagcaaactgagcgtggataaaagccgctggcagcgcggcgatacctttatttgcgcggtgatgcatgaagcgctgcataaccattatacccaggaaagcctgagccatagcccgggcaaacataaccattatacccaggaaagcctgagccatagcccgggcaaa

SEQ ID NO: 2 - protein, 215 aa, synthetic construct
  REGION 1..215: note = modified canine sequence
  VARIANT 4: note = misc_feature - Xaa can be any naturally occurring amino acid
  VARIANT 31: note = misc_feature - Xaa can be any naturally occurring amino acid
  VARIANT 63..65: note = misc_feature - Xaa can be any naturally occurring amino acid
  VARIANT 93: note = misc_feature - Xaa can be any naturally occurring amino acid
  VARIANT 95: note = misc_feature - Xaa can be any naturally occurring amino acid
LGGXSVFIFPPKPKDTLLIARTPEVTCVVVXLDPEDPEVQISWFVDGKQMQTAKTQPREEQFXXXYRVVSVLPIGHQDWLKGKQFTCKVNNKXLXSPIERTISKARGQAHQPSVYVLPPSREELSKNTVSLTCLIKDFFPPDIDVEWQSNGQQEPESKYRTTPPQLDEDGSYFLYSKLSVDKSRWQRGDTFICAVMHEALHNHYTQESLSHSPGK

SEQ ID NO: 3 - DNA, 690 bp, synthetic construct
  misc_feature 1..690: note = modified canine sequence
  misc_difference 10..12: note = n is a, c, g, or t
  misc_difference 91..93: note = n is a, c, g, or t
  misc_difference 187..195: note = n is a, c, g, or t
  misc_difference 277..279: note = n is a, c, g, or t
  misc_difference 283..285: note = n is a, c, g, or t
  source 1..690: mol_type = other DNA
ctgggcggcnnnagcgtgtttatttttccgccgaaaccgaaagatattctggtgaccgcgcgcaccccgaccgtgacctgcgtggtggtgnnnctggatccggaaaacccggaagtgcagattagctggtttgtggatagcaaacaggtgcagaccgcgaacacccagccgcgcgaagaacagagcnnnnnnnnntatcgcgtggtgagcgtgctgccgattggccatcaggattggctgagcggcaaacagtttaaatgcaaagtgaacaacaaannnctgnnnagcccgattgaagaaattattagcaaaaccccgggccaggcgcatcagccgaacgtgtatgtgctgccgccgagccgcgatgaaatgagcaaaaacaccgtgaccctgacctgcctggtgaaagatttttttccgccggaaattgatgtggaatggcagagcaacggccagcaggaaccggaaagcaaatatcgcatgaccccgccgcagctggatgaagatggcagctattttctgtatagcaaactgagcgtggataaaagccgctggcagcgcggcgatacctttatttgcgcggtgatgcatgaagcgctgcataaccattatacccagattagcctgagccatagcccgggcaaacataaccattatacccagattagcctgagccatagcccgggcaaa

SEQ ID NO: 4 - protein, 215 aa, synthetic construct
  REGION 1..215: note = modified canine sequence
  VARIANT 4: note = misc_feature - Xaa can be any naturally occurring amino acid
  VARIANT 31: note = misc_feature - Xaa can be any naturally occurring amino acid
  VARIANT 63..65: note = misc_feature - Xaa can be any naturally occurring amino acid
  VARIANT 93: note = misc_feature - Xaa can be any naturally occurring amino acid
  VARIANT 95: note = misc_feature - Xaa can be any naturally occurring amino acid
LGGXSVFIFPPKPKDILVTARTPTVTCVVVXLDPENPEVQISWFVDSKQVQTANTQPREEQSXXXYRVVSVLPIGHQDWLSGKQFKCKVNNKXLXSPIEEIISKTPGQAHQPNVYVLPPSRDEMSKNTVTLTCLVKDFFPPEIDVEWQSNGQQEPESKYRMTPPQLDEDGSYFLYSKLSVDKSRWQRGDTFICAVMHEALHNHYTQISLSHSPGK

SEQ ID NO: 5 - DNA, 699 bp, synthetic construct
  misc_feature 1..699: note = modified canine sequence
  source 1..699: mol_type = other DNA
ccgaaagaaagcacctgcaaatgcattccgccgtgcccggtgccggaaagcctgggcggcccgagcgtgtttatttttccgccgaaaccgaaagatattctgcgcattacccgcaccccggaaattacctgcgtggtgctggatctgggccgcgaagatccggaagtgcagattagctggtttgtggatggcaaagaagtgcataccgcgaaaacccagccgcgcgaacagcagtttaacagcacctatcgcgtggtgagcgtgctgccgattgaacatcaggattggctgaccggcaaagaatttaaatgccgcgtgaaccatattggcctgccgagcccgattgaacgcaccattagcaaagcgcgcggccaggcgcatcagccgagcgtgtatgtgctgccgccgagcccgaaagaactgagcagcagcgataccgtgaccctgacctgcctgattaaagatttttttccgccggaaattgatgtggaatggcagagcaacggccagccggaaccggaaagcaaatatcataccaccgcgccgcagctggatgaagatggcagctattttctgtatagcaaactgagcgtggataaaagccgctggcagcagggcgatacctttacctgcgcggtgatgcatgaagcgctgcagaaccattataccgatctgagcctgagccatagcccgggcaaa

SEQ ID NO: 6 - protein, 233 aa, synthetic construct
  REGION 1..233: note = modified canine sequence
PKESTCKCIPPCPVPESLGGPSVFIFPPKPKDILRITRTPEITCVVLDLGREDPEVQISWFVDGKEVHTAKTQPREQQFNSTYRVVSVLPIEHQDWLTGKEFKCRVNHIGLPSPIERTISKARGQAHQPSVYVLPPSPKELSSSDTVTLTCLIKDFFPPEIDVEWQSNGQPEPESKYHTTAPQLDEDGSYFLYSKLSVDKSRWQQGDTFTCAVMHEALQNHYTDLSLSHSPGK

SEQ ID NO: 7 - DNA, 699 bp, synthetic construct
  misc_feature 1..699: note = modified canine sequence
  source 1..699: mol_type = other DNA
tttaacgaatgccgctgcaccgataccccgccgtgcccggtgccggaaccgctgggcggcccgagcgtgtttatttttccgccgaaaccgaaagatattctgcgcattacccgcaccccggaaattacctgcgtggtgctggatctgggccgcgaagatccggaagtgcagattagctggtttgtggatggcaaagaagtgcataccgcgaaaacccagccgcgcgaacagcagtttaacagcacctatcgcgtggtgagcgtgctgccgattgaacatcaggattggctgaccggcaaagaatttaaatgccgcgtgaaccatattggcctgccgagcccgattgaacgcaccattagcaaagcgcgcggccaggcgcatcagccgagcgtgtatgtgctgccgccgagcccgaaagaactgagcagcagcgataccgtgaccctgacctgcctgattaaagatttttttccgccggaaattgatgtggaatggcagagcaacggccagccggaaccggaaagcaaatatcataccaccgcgccgcagctggatgaagatggcagctattttctgtatagcaaactgagcgtggataaaagccgctggcagcagggcgatacctttacctgcgcggtgatgcatgaagcgctgcagaaccattataccgatctgagcctgagccatagcccgggcaaa

SEQ ID NO: 8 - protein, 233 aa, synthetic construct
  REGION 1..233: note = modified canine sequence
FNECRCTDTPPCPVPEPLGGPSVFIFPPKPKDILRITRTPEITCVVLDLGREDPEVQISWFVDGKEVHTAKTQPREQQFNSTYRVVSVLPIEHQDWLTGKEFKCRVNHIGLPSPIERTISKARGQAHQPSVYVLPPSPKELSSSDTVTLTCLIKDFFPPEIDVEWQSNGQPEPESKYHTTAPQLDEDGSYFLYSKLSVDKSRWQQGDTFTCAVMHEALQNHYTDLSLSHSPGK

SEQ ID NO: 9 - DNA, 714 bp, synthetic construct
  misc_feature 1..714: note = modified canine sequence
  source 1..714: mol_type = other DNA
ccgaaacgcgaaaacggccgcgtgccgcgcccgccggattgcccgaaatgcccggcgccggaaatgctgggcggcccgagcgtgtttatttttccgccgaaaccgaaagatattctgcgcattacccgcaccccggaaattacctgcgtggtgctggatctgggccgcgaagatccggaagtgcagattagctggtttgtggatggcaaagaagtgcataccgcgaaaacccagccgcgcgaacagcagtttaacagcacctatcgcgtggtgagcgtgctgccgattgaacatcaggattggctgaccggcaaagaatttaaatgccgcgtgaaccatattggcctgccgagcccgattgaacgcaccattagcaaagcgcgcggccaggcgcatcagccgagcgtgtatgtgctgccgccgagcccgaaagaactgagcagcagcgataccgtgaccctgacctgcctgattaaagatttttttccgccggaaattgatgtggaatggcagagcaacggccagccggaaccggaaagcaaatatcataccaccgcgccgcagctggatgaagatggcagctattttctgtatagcaaactgagcgtggataaaagccgctggcagcagggcgatacctttacctgcgcggtgatgcatgaagcgctgcagaaccattataccgatctgagcctgagccatagcccgggcaaa

SEQ ID NO: 10 - protein, 238 aa, synthetic construct
  REGION 1..238: note = modified canine sequence
PKRENGRVPRPPDCPKCPAPEMLGGPSVFIFPPKPKDILRITRTPEITCVVLDLGREDPEVQISWFVDGKEVHTAKTQPREQQFNSTYRVVSVLPIEHQDWLTGKEFKCRVNHIGLPSPIERTISKARGQAHQPSVYVLPPSPKELSSSDTVTLTCLIKDFFPPEIDVEWQSNGQPEPESKYHTTAPQLDEDGSYFLYSKLSVDKSRWQQGDTFTCAVMHEALQNHYTDLSLSHSPGK

SEQ ID NO: 11 - DNA, 708 bp, synthetic construct
  misc_feature 1..708: note = modified canine sequence
  source 1..708: mol_type = other DNA
gccaaggagtgcgagtgcaagtgcaactgcaacaactgcccctgccccggctgcggcctgctgggcggccccagcgtgttcatcttcccccccaagcccaaggacatcctgagaatcaccagaacccccgagatcacctgcgtggtgctggacctgggcagagaggaccccgaggtgcagatcagctggttcgtggacggcaaggaggtgcacaccgccaagacccagcccagagagcagcagttcaacagcacctacagagtggtgagcgtgctgcccatcgagcaccaggactggctgaccggcaaggagttcaagtgcagagtgaaccacatcggcctgcccagccccatcgagagaaccatcagcaaggccagaggccaggcccaccagcccagcgtgtacgtgctgccccccagccccaaggagctgagcagcagcgacaccgtgaccctgacctgcctgatcaaggacttcttcccccccgagatcgacgtggagtggcagagcaacggccagcccgagcccgagagcaagtaccacaccaccgccccccagctggacgaggacggcagctacttcctgtacagcaagctgagcgtggacaagagcagatggcagcagggcgacaccttcacctgcgccgtgatgcacgaggccctgcagaaccactacaccgacctgagcctgagccacagccccggcaag

SEQ ID NO: 12 - protein, 236 aa, synthetic construct
  REGION 1..236: note = modified canine sequence
AKECECKCNCNNCPCPGCGLLGGPSVFIFPPKPKDILRITRTPEITCVVLDLGREDPEVQISWFVDGKEVHTAKTQPREQQFNSTYRVVSVLPIEHQDWLTGKEFKCRVNHIGLPSPIERTISKARGQAHQPSVYVLPPSPKELSSSDTVTLTCLIKDFFPPEIDVEWQSNGQPEPESKYHTTAPQLDEDGSYFLYSKLSVDKSRWQQGDTFTCAVMHEALQNHYTDLSLSHSPGK

SEQ ID NO: 13 - protein, 17 aa, Mus musculus
KSSQSLLNSVNQKNYLA

SEQ ID NO: 14 - protein, 16 aa, Mus musculus
RSSQNIVHSNGNTYLE

SEQ ID NO: 15 - protein, 11 aa, Mus musculus
HASQNINVWLS

SEQ ID NO: 16 - protein, 7 aa, Mus musculus
FASTRVS

SEQ ID NO: 17 - protein, 7 aa, Mus musculus
KVSNRFS

SEQ ID NO: 18 - protein, 7 aa, Mus musculus
KASHLHT

SEQ ID NO: 19 - protein, 7 aa, Mus musculus
FASARVS

SEQ ID NO: 20 - protein, 7 aa, Mus musculus
FASTRIS

SEQ ID NO: 21 - protein, 7 aa, Mus musculus
KASNLHT

SEQ ID NO: 22 - protein, 9 aa, Mus musculus
QQYFSTPLT

SEQ ID NO: 23 - protein, 9 aa, Mus musculus
FQGSHVPYT

SEQ ID NO: 24 - protein, 9 aa, Mus musculus
QQGQSWPLT

SEQ ID NO: 25 - protein, 9 aa, Mus musculus
QQYFSTPLT

SEQ ID NO: 26 - protein, 9 aa, Mus musculus
QQGQSYPLT

SEQ ID NO: 27 - protein, 10 aa, Mus musculus
GYTFTTYGMS

SEQ ID NO: 28 - protein, 10 aa, Mus musculus
GYTFTRYNMH

SEQ ID NO: 29 - protein, 10 aa, Mus musculus
GFNIKNTYMH

SEQ ID NO: 30 - protein, 10 aa, Mus musculus
GFSLTSYGVH

SEQ ID NO: 31 - protein, 17 aa, Mus musculus
WINIYSGIPTYADDFKG

SEQ ID NO: 32 - protein, 17 aa, Mus musculus
TIYPGYGDTSYNQKFKG

SEQ ID NO: 33 - protein, 17 aa, Mus musculus
RIAPANVDTKYAPKFQG

SEQ ID NO: 34 - protein, 17 aa, Mus musculus
WINIYSGMPTYADDFKG

SEQ ID NO: 35 - protein, 17 aa, Mus musculus
RIDPANVNTKYAPKFQG

SEQ ID NO: 36 - protein, 6 aa, Mus musculus
FDGPDY

SEQ ID NO: 37 - protein, 13 aa, Mus musculus
EFADDYPIPPFDY

SEQ ID NO: 38 - protein, 11 aa, Mus musculus
IYYDYDGDIDV

SEQ ID NO: 39 - DNA, 1350 bp, synthetic construct
  misc_feature 1..1350: note = caninized mouse antibody
  misc_difference 715..717: note = n is a, c, g, or t
  misc_difference 796..798: note = n is a, c, g, or t
  misc_difference 892..900: note = n is a, c, g, or t
  misc_difference 982..984: note = n is a, c, g, or t
  misc_difference 988..990: note = n is a, c, g, or t
  source 1..1350: mol_type = other DNA
gaggtgcagctggtgcagagcggcggcgacctggtgaagcccggcggcagcgtgagactgagctgcgtggccagcggctacaccttcaccacctacggcatgagctgggtgagacaggcccccggcaagggcctgcagtggatgggctggatcaacatctacagcggcatccccacctacgccgacgacttcaagggcagattcaccttcagcctggacaccgccaagaacaccgcctacctgcagctgaacagcctgagagccgaggacaccgccgtgtactactgcaccagattcgacggccccgactactggggccagggcaccctggtgaccgtgagcagcgccagcaccaccgcccccagcgtgttccccctggcccccagctgcggcagcaccagcggcagcaccgtggccctggcctgcctggtgagcggctacttccccgagcccgtgaccgtgagctggaacagcggcagcctgaccagcggcgtgcacaccttccccagcgtgctgcagagcagcggcctgtacagcctgagcagcatggtgaccgtgcccagcagcagatggcccagcgagaccttcacctgcaacgtggcccaccccgccagcaagaccaaggtggacaagcccgtgcccaagagagagaacggcagagtgcccagaccccccgactgccccaagtgccccgcccccgagatgctgggcggcnnnagcgtgttcatcttcccccccaagcccaaggacaccctgctgatcgccagaacccccgaggtgacctgcgtggtggtgnnnctggaccccgaggaccccgaggtgcagatcagctggttcgtggacggcaagcagatgcagaccgccaagacccagcccagagaggagcagttcnnnnnnnnntacagagtggtgagcgtgctgcccatcggccaccaggactggctgaagggcaagcagttcacctgcaaggtgaacaacaagnnnctgnnnagccccatcgagagaaccatcagcaaggccagaggccaggcccaccagcccagcgtgtacgtgctgccccccagcagagaggagctgagcaagaacaccgtgagcctgacctgcctgatcaaggacttcttcccccccgacatcgacgtggagtggcagagcaacggccagcaggagcccgagagcaagtacagaaccacccccccccagctggacgaggacggcagctacttcctgtacagcaagctgagcgtggacaagagcagatggcagagaggcgacaccttcatctgcgccgtgatgcacgaggccctgcacaaccactacacccaggagagcctgagccacagccccggcaag

SEQ ID NO: 40 - protein, 450 aa, synthetic construct
  REGION 1..450: note = caninized mouse antibody
  VARIANT 239: note = misc_feature - Xaa can be any naturally occurring amino acid
  VARIANT 266: note = misc_feature - Xaa can be any naturally occurring amino acid
  VARIANT 298..300: note = misc_feature - Xaa can be any naturally occurring amino acid
  VARIANT 328: note = misc_feature - Xaa can be any naturally occurring amino acid
  VARIANT 330: note = misc_feature - Xaa can be any naturally occurring amino acid
EVQLVQSGGDLVKPGGSVRLSCVASGYTFTTYGMSWVRQAPGKGLQWMGWINIYSGIPTYADDFKGRFTFSLDTAKNTAYLQLNSLRAEDTAVYYCTRFDGPDYWGQGTLVTVSSASTTAPSVFPLAPSCGSTSGSTVALACLVSGYFPEPVTVSWNSGSLTSGVHTFPSVLQSSGLYSLSSMVTVPSSRWPSETFTCNVAHPASKTKVDKPVPKRENGRVPRPPDCPKCPAPEMLGGXSVFIFPPKPKDTLLIARTPEVTCVVVXLDPEDPEVQISWFVDGKQMQTAKTQPREEQFXXXYRVVSVLPIGHQDWLKGKQFTCKVNNKXLXSPIERTISKARGQAHQPSVYVLPPSREELSKNTVSLTCLIKDFFPPDIDVEWQSNGQQEPESKYRTTPPQLDEDGSYFLYSKLSVDKSRWQRGDTFICAVMHEALHNHYTQESLSHSPGK

SEQ ID NO: 41 - DNA, 1344 bp, synthetic construct
  misc_feature 1..1344: note = caninized mouse antibody
  misc_difference 709..711: note = n is a, c, g, or t
  misc_difference 790..792: note = n is a, c, g, or t
  misc_difference 886..894: note = n is a, c, g, or t
  misc_difference 976..978: note = n is a, c, g, or t
  misc_difference 982..984: note = n is a, c, g, or t
  source 1..1344: mol_type = other DNA
gaggtgcagctggtgcagagcggcggcgacctggtgaagcccggcggcagcgtgagactgagctgcgtggccagcggctacaccttcaccacctacggcatgagctgggtgagacaggcccccggcaagggcctgcagtggatgggctggatcaacatctacagcggcatccccacctacgccgacgacttcaagggcagattcaccttcagcctggacaccgccaagaacaccgcctacctgcagctgaacagcctgagagccgaggacaccgccgtgtactactgcaccagattcgacggccccgactactggggccagggcaccctggtgaccgtgagcagcgccagcaccaccgcccccagcgtgttccccctggcccccagctgcggcagccagagcggcagcaccgtggccctggcctgcctggtgagcggctacatccccgagcccgtgaccgtgagctggaacagcgtgagcctgaccagcggcgtgcacaccttccccagcgtgctgcagagcagcggcctgtacagcctgagcagcatggtgaccgtgcccagcagcagatggcccagcgagaccttcacctgcaacgtggcccaccccgccaccaacaccaaggtggacaagcccgtggccaaggagtgcgagtgcaagtgcaactgcaacaactgcccctgccccggctgcggcctgctgggcggcnnnagcgtgttcatcttcccccccaagcccaaggacatcctggtgaccgccagaacccccaccgtgacctgcgtggtggtgnnnctggaccccgagaaccccgaggtgcagatcagctggttcgtggacagcaagcaggtgcagaccgccaacacccagcccagagaggagcagagcnnnnnnnnntacagagtggtgagcgtgctgcccatcggccaccaggactggctgagcggcaagcagttcaagtgcaaggtgaacaacaagnnnctgnnnagccccatcgaggagatcatcagcaagacccccggccaggcccaccagcccaacgtgtacgtgctgccccccagcagagacgagatgagcaagaacaccgtgaccctgacctgcctggtgaaggacttcttcccccccgagatcgacgtggagtggcagagcaacggccagcaggagcccgagagcaagtacagaatgacccccccccagctggacgaggacggcagctacttcctgtacagcaagctgagcgtggacaagagcagatggcagagaggcgacaccttcatctgcgccgtgatgcacgaggccctgcacaaccactacacccagatcagcctgagccacagccccggcaag

SEQ ID NO: 42 - protein, 448 aa, synthetic construct
  REGION 1..448: note = caninized mouse antibody
  VARIANT 237: note = misc_feature - Xaa can be any naturally occurring amino acid
  VARIANT 264: note = misc_feature - Xaa can be any naturally occurring amino acid
  VARIANT 296..298: note = misc_feature - Xaa can be any naturally occurring amino acid
  VARIANT 326: note = misc_feature - Xaa can be any naturally occurring amino acid
  VARIANT 328: note = misc_feature - Xaa can be any naturally occurring amino acid
EVQLVQSGGDLVKPGGSVRLSCVASGYTFTTYGMSWVRQAPGKGLQWMGWINIYSGIPTYADDFKGRFTFSLDTAKNTAYLQLNSLRAEDTAVYYCTRFDGPDYWGQGTLVTVSSASTTAPSVFPLAPSCGSQSGSTVALACLVSGYIPEPVTVSWNSVSLTSGVHTFPSVLQSSGLYSLSSMVTVPSSRWPSETFTCNVAHPATNTKVDKPVAKECECKCNCNNCPCPGCGLLGGXSVFIFPPKPKDILVTARTPTVTCVVVXLDPENPEVQISWFVDSKQVQTANTQPREEQSXXXYRVVSVLPIGHQDWLSGKQFKCKVNNKXLXSPIEEIISKTPGQAHQPNVYVLPPSRDEMSKNTVTLTCLVKDFFPPEIDVEWQSNGQQEPESKYRMTPPQLDEDGSYFLYSKLSVDKSRWQRGDTFICAVMHEALHNHYTQISLSHSPGK

SEQ ID NO: 43 - DNA, 1365 bp, synthetic construct
  misc_feature 1..1365: note = caninized mouse antibody
  misc_difference 730..732: note = n is a, c, g, or t
  misc_difference 811..813: note = n is a, c, g, or t
  misc_difference 907..915: note = n is a, c, g, or t
  misc_difference 997..999: note = n is a, c, g, or t
  misc_difference 1003..1005: note = n is a, c, g, or t
  source 1..1365: mol_type = other DNA
gaggtgcagctggtgcagagcggcggcgacctggtgaagcccggcggcagcgtgagactgagctgcgtggccagcggcttcaacatcaagaacacctacatgcactgggtgagacaggcccccggcaagggcctgcagtggatcggcagaatcgcccccgccaacgtggacaccaagtacgcccccaagttccagggcaaggccaccatcagcgccgacaccgccaagaacaccgcctacatgcagctgaacagcctgagagccgaggacaccgccgtgtactactgcgtgctgatctactacgactacgacggcgacatcgacgtgtggggccagggcaccctggtgaccgtgagcagcgccagcaccaccgcccccagcgtgttccccctggcccccagctgcggcagcaccagcggcagcaccgtggccctggcctgcctggtgagcggctacttccccgagcccgtgaccgtgagctggaacagcggcagcctgaccagcggcgtgcacaccttccccagcgtgctgcagagcagcggcctgtacagcctgagcagcatggtgaccgtgcccagcagcagatggcccagcgagaccttcacctgcaacgtggcccaccccgccagcaagaccaaggtggacaagcccgtgcccaagagagagaacggcagagtgcccagaccccccgactgccccaagtgccccgcccccgagatgctgggcggcnnnagcgtgttcatcttcccccccaagcccaaggacaccctgctgatcgccagaacccccgaggtgacctgcgtggtggtgnnnctggaccccgaggaccccgaggtgcagatcagctggttcgtggacggcaagcagatgcagaccgccaagacccagcccagagaggagcagttcnnnnnnnnntacagagtggtgagcgtgctgcccatcggccaccaggactggctgaagggcaagcagttcacctgcaaggtgaacaacaagnnnctgnnnagccccatcgagagaaccatcagcaaggccagaggccaggcccaccagcccagcgtgtacgtgctgccccccagcagagaggagctgagcaagaacaccgtgagcctgacctgcctgatcaaggacttcttcccccccgacatcgacgtggagtggcagagcaacggccagcaggagcccgagagcaagtacagaaccacccccccccagctggacgaggacggcagctacttcctgtacagcaagctgagcgtggacaagagcagatggcagagaggcgacaccttcatctgcgccgtgatgcacgaggccctgcacaaccactacacccaggagagcctgagccacagccccggcaag

SEQ ID NO: 44 - protein, 455 aa, synthetic construct
  REGION 1..455: note = caninized mouse antibody
  VARIANT 244: note = misc_feature - Xaa can be any naturally occurring amino acid
  VARIANT 271: note = misc_feature - Xaa can be any naturally occurring amino acid
  VARIANT 303..305: note = misc_feature - Xaa can be any naturally occurring amino acid
  VARIANT 333: note = misc_feature - Xaa can be any naturally occurring amino acid
  VARIANT 335: note = misc_feature - Xaa can be any naturally occurring amino acid
EVQLVQSGGDLVKPGGSVRLSCVASGFNIKNTYMHWVRQAPGKGLQWIGRIAPANVDTKYAPKFQGKATISADTAKNTAYMQLNSLRAEDTAVYYCVLIYYDYDGDIDVWGQGTLVTVSSASTTAPSVFPLAPSCGSTSGSTVALACLVSGYFPEPVTVSWNSGSLTSGVHTFPSVLQSSGLYSLSSMVTVPSSRWPSETFTCNVAHPASKTKVDKPVPKRENGRVPRPPDCPKCPAPEMLGGXSVFIFPPKPKDTLLIARTPEVTCVVVXLDPEDPEVQISWFVDGKQMQTAKTQPREEQFXXXYRVVSVLPIGHQDWLKGKQFTCKVNNKXLXSPIERTISKARGQAHQPSVYVLPPSREELSKNTVSLTCLIKDFFPPDIDVEWQSNGQQEPESKYRTTPPQLDEDGSYFLYSKLSVDKSRWQRGDTFICAVMHEALHNHYTQESLSHSPGK

SEQ ID NO: 45 - DNA, 1359 bp, synthetic construct
  misc_feature 1..1359: note = caniinized mouse antibody
  misc_difference 724..726: note = n is a, c, g, or t
  misc_difference 805..807: note = n is a, c, g, or t
  misc_difference 901..909: note = n is a, c, g, or t
  misc_difference 991..993: note = n is a, c, g, or t
  misc_difference 997..999: note = n is a, c, g, or t
  source 1..1359: mol_type = other DNA
gaggtgcagctggtgcagagcggcggcgacctggtgaagcccggcggcagcgtgagactgagctgcgtggccagcggcttcaacatcaagaacacctacatgcactgggtgagacaggcccccggcaagggcctgcagtggatcggcagaatcgcccccgccaacgtggacaccaagtacgcccccaagttccagggcaaggccaccatcagcgccgacaccgccaagaacaccgcctacatgcagctgaacagcctgagagccgaggacaccgccgtgtactactgcgtgctgatctactacgactacgacggcgacatcgacgtgtggggccagggcaccctggtgaccgtgagcagcgccagcaccaccgcccccagcgtgttccccctggcccccagctgcggcagccagagcggcagcaccgtggccctggcctgcctggtgagcggctacatccccgagcccgtgaccgtgagctggaacagcgtgagcctgaccagcggcgtgcacaccttccccagcgtgctgcagagcagcggcctgtacagcctgagcagcatggtgaccgtgcccagcagcagatggcccagcgagaccttcacctgcaacgtggcccaccccgccaccaacaccaaggtggacaagcccgtggccaaggagtgcgagtgcaagtgcaactgcaacaactgcccctgccccggctgcggcctgctgggcggcnnnagcgtgttcatcttcccccccaagcccaaggacatcctggtgaccgccagaacccccaccgtgacctgcgtggtggtgnnnctggaccccgagaaccccgaggtgcagatcagctggttcgtggacagcaagcaggtgcagaccgccaacacccagcccagagaggagcagagcnnnnnnnnntacagagtggtgagcgtgctgcccatcggccaccaggactggctgagcggcaagcagttcaagtgcaaggtgaacaacaagnnnctgnnnagccccatcgaggagatcatcagcaagacccccggccaggcccaccagcccaacgtgtacgtgctgccccccagcagagacgagatgagcaagaacaccgtgaccctgacctgcctggtgaaggacttcttcccccccgagatcgacgtggagtggcagagcaacggccagcaggagcccgagagcaagtacagaatgacccccccccagctggacgaggacggcagctacttcctgtacagcaagctgagcgtggacaagagcagatggcagagaggcgacaccttcatctgcgccgtgatgcacgaggccctgcacaaccactacacccagatcagcctgagccacagccccggcaag

SEQ ID NO: 46 - protein, 453 aa, synthetic construct
  REGION 1..453: note = caninized mouse antibody
  VARIANT 242: note = misc_feature - Xaa can be any naturally occurring amino acid
  VARIANT 269: note = misc_feature - Xaa can be any naturally occurring amino acid
  VARIANT 301..303: note = misc_feature - Xaa can be any naturally occurring amino acid
  VARIANT 331: note = misc_feature - Xaa can be any naturally occurring amino acid
  VARIANT 333: note = misc_feature - Xaa can be any naturally occurring amino acid
EVQLVQSGGDLVKPGGSVRLSCVASGFNIKNTYMHWVRQAPGKGLQWIGRIAPANVDTKYAPKFQGKATISADTAKNTAYMQLNSLRAEDTAVYYCVLIYYDYDGDIDVWGQGTLVTVSSASTTAPSVFPLAPSCGSQSGSTVALACLVSGYIPEPVTVSWNSVSLTSGVHTFPSVLQSSGLYSLSSMVTVPSSRWPSETFTCNVAHPATNTKVDKPVAKECECKCNCNNCPCPGCGLLGGXSVFIFPPKPKDILVTARTPTVTCVVVXLDPENPEVQISWFVDSKQVQTANTQPREEQSXXXYRVVSVLPIGHQDWLSGKQFKCKVNNKXLXSPIEEIISKTPGQAHQPNVYVLPPSRDEMSKNTVTLTCLVKDFFPPEIDVEWQSNGQQEPESKYRMTPPQLDEDGSYFLYSKLSVDKSRWQRGDTFICAVMHEALHNHYTQISLSHSPGK

SEQ ID NO: 47 - DNA, 1371 bp, synthetic construct
  misc_feature 1..1371: note = caninized mouse antibody
  misc_difference 736..738: note = n is a, c, g, or t
  misc_difference 817..819: note = n is a, c, g, or t
  misc_difference 913..921: note = n is a, c, g, or t
  misc_difference 1003..1005: note = n is a, c, g, or t
  misc_difference 1009..1011: note = n is a, c, g, or t
  source 1..1371: mol_type = other DNA
gaggtgcagctggtgcagagcggcggcgacctggtgaagcccggcggcagcgtgagactgagctgcgtggccagcggctacaccttcaccagatacaacatgcactgggtgagacaggcccccggcaagggcctgcagtggatcggcaccatctaccccggctacggcgacaccagctacaaccagaagttcaagggcaaggccaccctgagcgtggacatcgccaagaacaccgcctacatgcagctgaacagcctgagagccgaggacaccgccgtgtacttctgcagcagagagttcgccgacgactaccccatcccccccttcgactactggggccagggcaccctggtgaccgtgagcagcgccagcaccaccgcccccagcgtgttccccctggcccccagctgcggcagcaccagcggcagcaccgtggccctggcctgcctggtgagcggctacttccccgagcccgtgaccgtgagctggaacagcggcagcctgaccagcggcgtgcacaccttccccagcgtgctgcagagcagcggcctgtacagcctgagcagcatggtgaccgtgcccagcagcagatggcccagcgagaccttcacctgcaacgtggcccaccccgccagcaagaccaaggtggacaagcccgtgcccaagagagagaacggcagagtgcccagaccccccgactgccccaagtgccccgcccccgagatgctgggcggcnnnagcgtgttcatcttcccccccaagcccaaggacaccctgctgatcgccagaacccccgaggtgacctgcgtggtggtgnnnctggaccccgaggaccccgaggtgcagatcagctggttcgtggacggcaagcagatgcagaccgccaagacccagcccagagaggagcagttcnnnnnnnnntacagagtggtgagcgtgctgcccatcggccaccaggactggctgaagggcaagcagttcacctgcaaggtgaacaacaagnnnctgnnnagccccatcgagagaaccatcagcaaggccagaggccaggcccaccagcccagcgtgtacgtgctgccccccagcagagaggagctgagcaagaacaccgtgagcctgacctgcctgatcaaggacttcttcccccccgacatcgacgtggagtggcagagcaacggccagcaggagcccgagagcaagtacagaaccacccccccccagctggacgaggacggcagctacttcctgtacagcaagctgagcgtggacaagagcagatggcagagaggcgacaccttcatctgcgccgtgatgcacgaggccctgcacaaccactacacccaggagagcctgagccacagccccggcaag

SEQ ID NO: 48 - protein, 457 aa, synthetic construct
  REGION 1..457: note = caninized mouse antibody
  VARIANT 246: note = misc_feature - Xaa can be any naturally occurring amino acid
  VARIANT 273: note = misc_feature - Xaa can be any naturally occurring amino acid
  VARIANT 305..307: note = misc_feature - Xaa can be any naturally occurring amino acid
  VARIANT 335: note = misc_feature - Xaa can be any naturally occurring amino acid
  VARIANT 337: note = misc_feature - Xaa can be any naturally occurring amino acid
EVQLVQSGGDLVKPGGSVRLSCVASGYTFTRYNMHWVRQAPGKGLQWIGTIYPGYGDTSYNQKFKGKATLSVDIAKNTAYMQLNSLRAEDTAVYFCSREFADDYPIPPFDYWGQGTLVTVSSASTTAPSVFPLAPSCGSTSGSTVALACLVSGYFPEPVTVSWNSGSLTSGVHTFPSVLQSSGLYSLSSMVTVPSSRWPSETFTCNVAHPASKTKVDKPVPKRENGRVPRPPDCPKCPAPEMLGGXSVFIFPPKPKDTLLIARTPEVTCVVVXLDPEDPEVQISWFVDGKQMQTAKTQPREEQFXXXYRVVSVLPIGHQDWLKGKQFTCKVNNKXLXSPIERTISKARGQAHQPSVYVLPPSREELSKNTVSLTCLIKDFFPPDIDVEWQSNGQQEPESKYRTTPPQLDEDGSYFLYSKLSVDKSRWQRGDTFICAVMHEALHNHYTQESLSHSPGK

SEQ ID NO: 49 - DNA, 1365 bp, synthetic construct
  misc_feature 1..1365: note = caninized mouse antibody
  misc_difference 730..732: note = n is a, c, g, or t
  misc_difference 811..813: note = n is a, c, g, or t
  misc_difference 907..915: note = n is a, c, g, or t
  misc_difference 997..999: note = n is a, c, g, or t
  misc_difference 1003..1005: note = n is a, c, g, or t
  source 1..1365: mol_type = other DNA
gaggtgcagctggtgcagagcggcggcgacctggtgaagcccggcggcagcgtgagactgagctgcgtggccagcggctacaccttcaccagatacaacatgcactgggtgagacaggcccccggcaagggcctgcagtggatcggcaccatctaccccggctacggcgacaccagctacaaccagaagttcaagggcaaggccaccctgagcgtggacatcgccaagaacaccgcctacatgcagctgaacagcctgagagccgaggacaccgccgtgtacttctgcagcagagagttcgccgacgactaccccatcccccccttcgactactggggccagggcaccctggtgaccgtgagcagcgccagcaccaccgcccccagcgtgttccccctggcccccagctgcggcagccagagcggcagcaccgtggccctggcctgcctggtgagcggctacatccccgagcccgtgaccgtgagctggaacagcgtgagcctgaccagcggcgtgcacaccttccccagcgtgctgcagagcagcggcctgtacagcctgagcagcatggtgaccgtgcccagcagcagatggcccagcgagaccttcacctgcaacgtggcccaccccgccaccaacaccaaggtggacaagcccgtggccaaggagtgcgagtgcaagtgcaactgcaacaactgcccctgccccggctgcggcctgctgggcggcnnnagcgtgttcatcttcccccccaagcccaaggacatcctggtgaccgccagaacccccaccgtgacctgcgtggtggtgnnnctggaccccgagaaccccgaggtgcagatcagctggttcgtggacagcaagcaggtgcagaccgccaacacccagcccagagaggagcagagcnnnnnnnnntacagagtggtgagcgtgctgcccatcggccaccaggactggctgagcggcaagcagttcaagtgcaaggtgaacaacaagnnnctgnnnagccccatcgaggagatcatcagcaagacccccggccaggcccaccagcccaacgtgtacgtgctgccccccagcagagacgagatgagcaagaacaccgtgaccctgacctgcctggtgaaggacttcttcccccccgagatcgacgtggagtggcagagcaacggccagcaggagcccgagagcaagtacagaatgacccccccccagctggacgaggacggcagctacttcctgtacagcaagctgagcgtggacaagagcagatggcagagaggcgacaccttcatctgcgccgtgatgcacgaggccctgcacaaccactacacccagatcagcctgagccacagccccggcaag

SEQ ID NO: 50 - protein, 455 aa, synthetic construct
  REGION 1..455: note = caninized mouse antibody
  VARIANT 244: note = misc_feature - Xaa can be any naturally occurring amino acid
  VARIANT 271: note = misc_feature - Xaa can be any naturally occurring amino acid
  VARIANT 303..305: note = misc_feature - Xaa can be any naturally occurring amino acid
  VARIANT 333: note = misc_feature - Xaa can be any naturally occurring amino acid
  VARIANT 335: note = misc_feature - Xaa can be any naturally occurring amino acid
EVQLVQSGGDLVKPGGSVRLSCVASGYTFTRYNMHWVRQAPGKGLQWIGTIYPGYGDTSYNQKFKGKATLSVDIAKNTAYMQLNSLRAEDTAVYFCSREFADDYPIPPFDYWGQGTLVTVSSASTTAPSVFPLAPSCGSQSGSTVALACLVSGYIPEPVTVSWNSVSLTSGVHTFPSVLQSSGLYSLSSMVTVPSSRWPSETFTCNVAHPATNTKVDKPVAKECECKCNCNNCPCPGCGLLGGXSVFIFPPKPKDILVTARTPTVTCVVVXLDPENPEVQISWFVDSKQVQTANTQPREEQSXXXYRVVSVLPIGHQDWLSGKQFKCKVNNKXLXSPIEEIISKTPGQAHQPNVYVLPPSRDEMSKNTVTLTCLVKDFFPPEIDVEWQSNGQQEPESKYRMTPPQLDEDGSYFLYSKLSVDKSRWQRGDTFICAVMHEALHNHYTQISLSHSPGK

SEQ ID NO: 51 - DNA, 1350 bp, synthetic construct
  misc_feature 1..1350: note = caninized mouse antibody
  misc_difference 715..717: note = n is a, c, g, or t
  misc_difference 796..798: note = n is a, c, g, or t
  misc_difference 892..900: note = n is a, c, g, or t
  misc_difference 982..984: note = n is a, c, g, or t
  misc_difference 988..990: note = n is a, c, g, or t
  source 1..1350: mol_type = other DNA
gaggtgcagctggtgcagagcggccccggcctggtgaagcccagccagagcctgagcctgacctgcgtggtgagcggcttcagcctgaccagctacggcgtgcactgggtgagacaggcccccggcaagggcctgcagtggatgggctggatcaacatctacagcggcatccccacctacgccgacgacttcaagggcagattcaccttcagcctggacaccgccaagaacaccgcctacctgcagctgagcagcctgagagccgaggacaccgccgtgtactactgcgccagattcgacggccccgactactggggccagggcaccctggtgaccgtgagcagcgccagcaccaccgcccccagcgtgttccccctggcccccagctgcggcagcaccagcggcagcaccgtggccctggcctgcctggtgagcggctacttccccgagcccgtgaccgtgagctggaacagcggcagcctgaccagcggcgtgcacaccttccccagcgtgctgcagagcagcggcctgtacagcctgagcagcatggtgaccgtgcccagcagcagatggcccagcgagaccttcacctgcaacgtggcccaccccgccagcaagaccaaggtggacaagcccgtgcccaagagagagaacggcagagtgcccagaccccccgactgccccaagtgccccgcccccgagatgctgggcggcnnnagcgtgttcatcttcccccccaagcccaaggacaccctgctgatcgccagaacccccgaggtgacctgcgtggtggtgnnnctggaccccgaggaccccgaggtgcagatcagctggttcgtggacggcaagcagatgcagaccgccaagacccagcccagagaggagcagttcnnnnnnnnntacagagtggtgagcgtgctgcccatcggccaccaggactggctgaagggcaagcagttcacctgcaaggtgaacaacaagnnnctgnnnagccccatcgagagaaccatcagcaaggccagaggccaggcccaccagcccagcgtgtacgtgctgccccccagcagagaggagctgagcaagaacaccgtgagcctgacctgcctgatcaaggacttcttcccccccgacatcgacgtggagtggcagagcaacggccagcaggagcccgagagcaagtacagaaccacccccccccagctggacgaggacggcagctacttcctgtacagcaagctgagcgtggacaagagcagatggcagagaggcgacaccttcatctgcgccgtgatgcacgaggccctgcacaaccactacacccaggagagcctgagccacagccccggcaag

SEQ ID NO: 52 - protein, 450 aa, synthetic construct
  REGION 1..450: note = caninized mouse antibody
  VARIANT 239: note = misc_feature - Xaa can be any naturally occurring amino acid
  VARIANT 266: note = misc_feature - Xaa can be any naturally occurring amino acid
  VARIANT 298..300: note = misc_feature - Xaa can be any naturally occurring amino acid
  VARIANT 328: note = misc_feature - Xaa can be any naturally occurring amino acid
  VARIANT 330: note = misc_feature - Xaa can be any naturally occurring amino acid
EVQLVQSGPGLVKPSQSLSLTCVVSGFSLTSYGVHWVRQAPGKGLQWMGWINIYSGIPTYADDFKGRFTFSLDTAKNTAYLQLSSLRAEDTAVYYCARFDGPDYWGQGTLVTVSSASTTAPSVFPLAPSCGSTSGSTVALACLVSGYFPEPVTVSWNSGSLTSGVHTFPSVLQSSGLYSLSSMVTVPSSRWPSETFTCNVAHPASKTKVDKPVPKRENGRVPRPPDCPKCPAPEMLGGXSVFIFPPKPKDTLLIARTPEVTCVVVXLDPEDPEVQISWFVDGKQMQTAKTQPREEQFXXXYRVVSVLPIGHQDWLKGKQFTCKVNNKXLXSPIERTISKARGQAHQPSVYVLPPSREELSKNTVSLTCLIKDFFPPDIDVEWQSNGQQEPESKYRTTPPQLDEDGSYFLYSKLSVDKSRWQRGDTFICAVMHEALHNHYTQESLSHSPGK

SEQ ID NO: 53 - DNA, 1344 bp, synthetic construct
  misc_feature 1..1344: note = caninized mouse antibody
  misc_difference 709..711: note = n is a, c, g, or t
  misc_difference 790..792: note = n is a, c, g, or t
  misc_difference 886..894: note = n is a, c, g, or t
  misc_difference 976..978: note = n is a, c, g, or t
  misc_difference 982..984: note = n is a, c, g, or t
  source 1..1344: mol_type = other DNA
gaggtgcagctggtgcagagcggccccggcctggtgaagcccagccagagcctgagcctgacctgcgtggtgagcggcttcagcctgaccagctacggcgtgcactgggtgagacaggcccccggcaagggcctgcagtggatgggctggatcaacatctacagcggcatccccacctacgccgacgacttcaagggcagattcaccttcagcctggacaccgccaagaacaccgcctacctgcagctgagcagcctgagagccgaggacaccgccgtgtactactgcgccagattcgacggccccgactactggggccagggcaccctggtgaccgtgagcagcgccagcaccaccgcccccagcgtgttccccctggcccccagctgcggcagccagagcggcagcaccgtggccctggcctgcctggtgagcggctacatccccgagcccgtgaccgtgagctggaacagcgtgagcctgaccagcggcgtgcacaccttccccagcgtgctgcagagcagcggcctgtacagcctgagcagcatggtgaccgtgcccagcagcagatggcccagcgagaccttcacctgcaacgtggcccaccccgccaccaacaccaaggtggacaagcccgtggccaaggagtgcgagtgcaagtgcaactgcaacaactgcccctgccccggctgcggcctgctgggcggcnnnagcgtgttcatcttcccccccaagcccaaggacatcctggtgaccgccagaacccccaccgtgacctgcgtggtggtgnnnctggaccccgagaaccccgaggtgcagatcagctggttcgtggacagcaagcaggtgcagaccgccaacacccagcccagagaggagcagagcnnnnnnnnntacagagtggtgagcgtgctgcccatcggccaccaggactggctgagcggcaagcagttcaagtgcaaggtgaacaacaagnnnctgnnnagccccatcgaggagatcatcagcaagacccccggccaggcccaccagcccaacgtgtacgtgctgccccccagcagagacgagatgagcaagaacaccgtgaccctgacctgcctggtgaaggacttcttcccccccgagatcgacgtggagtggcagagcaacggccagcaggagcccgagagcaagtacagaatgacccccccccagctggacgaggacggcagctacttcctgtacagcaagctgagcgtggacaagagcagatggcagagaggcgacaccttcatctgcgccgtgatgcacgaggccctgcacaaccactacacccagatcagcctgagccacagccccggcaag

SEQ ID NO: 54 - protein, 448 aa, synthetic construct
  REGION 1..448: note = caninized mouse antibody
  VARIANT 237: note = misc_feature - Xaa can be any naturally occurring amino acid
  VARIANT 264: note = misc_feature - Xaa can be any naturally occurring amino acid
  VARIANT 296..298: note = misc_feature - Xaa can be any naturally occurring amino acid
  VARIANT 326: note = misc_feature - Xaa can be any naturally occurring amino acid
  VARIANT 328: note = misc_feature - Xaa can be any naturally occurring amino acid
EVQLVQSGPGLVKPSQSLSLTCVVSGFSLTSYGVHWVRQAPGKGLQWMGWINIYSGIPTYADDFKGRFTFSLDTAKNTAYLQLSSLRAEDTAVYYCARFDGPDYWGQGTLVTVSSASTTAPSVFPLAPSCGSQSGSTVALACLVSGYIPEPVTVSWNSVSLTSGVHTFPSVLQSSGLYSLSSMVTVPSSRWPSETFTCNVAHPATNTKVDKPVAKECECKCNCNNCPCPGCGLLGGXSVFIFPPKPKDILVTARTPTVTCVVVXLDPENPEVQISWFVDSKQVQTANTQPREEQSXXXYRVVSVLPIGHQDWLSGKQFKCKVNNKXLXSPIEEIISKTPGQAHQPNVYVLPPSRDEMSKNTVTLTCLVKDFFPPEIDVEWQSNGQQEPESKYRMTPPQLDEDGSYFLYSKLSVDKSRWQRGDTFICAVMHEALHNHYTQISLSHSPGK

SEQ ID NO: 55 - DNA, 1350 bp, synthetic construct
  misc_feature 1..1350: note = caninized mouse antidody
  misc_difference 715..717: note = n is a, c, g, or t
  misc_difference 796..798: note = n is a, c, g, or t
  misc_difference 892..900: note = n is a, c, g, or t
  misc_difference 982..984: note = n is a, c, g, or t
  misc_difference 988..990: note = n is a, c, g, or t
  source 1..1350: mol_type = other DNA
gaggtgcagctggtgcagagcggcgccgaggtgaagaagcccggcgccagcgtgaaggtgagctgcaaggccagcggctacaccttcaccacctacggcatgagctgggtgagacaggcccccggcaagggcctgcagtggatgggctggatcaacatctacagcggcatccccacctacgccgacgacttcaagggcagattcgccctgagcctggacaccagcaccagcaccgcctacatggagctgaacagcctgagagccgaggacaccgccgtgtactactgcgccagattcgacggccccgactactggggccagggcaccctggtgaccgtgagcagcgccagcaccaccgcccccagcgtgttccccctggcccccagctgcggcagcaccagcggcagcaccgtggccctggcctgcctggtgagcggctacttccccgagcccgtgaccgtgagctggaacagcggcagcctgaccagcggcgtgcacaccttccccagcgtgctgcagagcagcggcctgtacagcctgagcagcatggtgaccgtgcccagcagcagatggcccagcgagaccttcacctgcaacgtggcccaccccgccagcaagaccaaggtggacaagcccgtgcccaagagagagaacggcagagtgcccagaccccccgactgccccaagtgccccgcccccgagatgctgggcggcnnnagcgtgttcatcttcccccccaagcccaaggacaccctgctgatcgccagaacccccgaggtgacctgcgtggtggtgnnnctggaccccgaggaccccgaggtgcagatcagctggttcgtggacggcaagcagatgcagaccgccaagacccagcccagagaggagcagttcnnnnnnnnntacagagtggtgagcgtgctgcccatcggccaccaggactggctgaagggcaagcagttcacctgcaaggtgaacaacaagnnnctgnnnagccccatcgagagaaccatcagcaaggccagaggccaggcccaccagcccagcgtgtacgtgctgccccccagcagagaggagctgagcaagaacaccgtgagcctgacctgcctgatcaaggacttcttcccccccgacatcgacgtggagtggcagagcaacggccagcaggagcccgagagcaagtacagaaccacccccccccagctggacgaggacggcagctacttcctgtacagcaagctgagcgtggacaagagcagatggcagagaggcgacaccttcatctgcgccgtgatgcacgaggccctgcacaaccactacacccaggagagcctgagccacagccccggcaag

SEQ ID NO: 56 - protein, 450 aa, synthetic construct
  REGION 1..450: note = caninized mouse antibody
  VARIANT 239: note = misc_feature - Xaa can be any naturally occurring amino acid
  VARIANT 266: note = misc_feature - Xaa can be any naturally occurring amino acid
  VARIANT 298..300: note = misc_feature - Xaa can be any naturally occurring amino acid
  VARIANT 328: note = misc_feature - Xaa can be any naturally occurring amino acid
  VARIANT 330: note = misc_feature - Xaa can be any naturally occurring amino acid
EVQLVQSGAEVKKPGASVKVSCKASGYTFTTYGMSWVRQAPGKGLQWMGWINIYSGIPTYADDFKGRFALSLDTSTSTAYMELNSLRAEDTAVYYCARFDGPDYWGQGTLVTVSSASTTAPSVFPLAPSCGSTSGSTVALACLVSGYFPEPVTVSWNSGSLTSGVHTFPSVLQSSGLYSLSSMVTVPSSRWPSETFTCNVAHPASKTKVDKPVPKRENGRVPRPPDCPKCPAPEMLGGXSVFIFPPKPKDTLLIARTPEVTCVVVXLDPEDPEVQISWFVDGKQMQTAKTQPREEQFXXXYRVVSVLPIGHQDWLKGKQFTCKVNNKXLXSPIERTISKARGQAHQPSVYVLPPSREELSKNTVSLTCLIKDFFPPDIDVEWQSNGQQEPESKYRTTPPQLDEDGSYFLYSKLSVDKSRWQRGDTFICAVMHEALHNHYTQESLSHSPGK

SEQ ID NO: 57 - DNA, 1344 bp, synthetic construct
  misc_feature 1..1344: note = caninized mouse antibody
  misc_difference 709..711: note = n is a, c, g, or t
  misc_difference 790..792: note = n is a, c, g, or t
  misc_difference 886..894: note = n is a, c, g, or t
  misc_difference 976..978: note = n is a, c, g, or t
  misc_difference 982..984: note = n is a, c, g, or t
  source 1..1344: mol_type = other DNA
gaggtgcagctggtgcagagcggcgccgaggtgaagaagcccggcgccagcgtgaaggtgagctgcaaggccagcggctacaccttcaccacctacggcatgagctgggtgagacaggcccccggcaagggcctgcagtggatgggctggatcaacatctacagcggcatccccacctacgccgacgacttcaagggcagattcgccctgagcctggacaccagcaccagcaccgcctacatggagctgaacagcctgagagccgaggacaccgccgtgtactactgcgccagattcgacggccccgactactggggccagggcaccctggtgaccgtgagcagcgccagcaccaccgcccccagcgtgttccccctggcccccagctgcggcagccagagcggcagcaccgtggccctggcctgcctggtgagcggctacatccccgagcccgtgaccgtgagctggaacagcgtgagcctgaccagcggcgtgcacaccttccccagcgtgctgcagagcagcggcctgtacagcctgagcagcatggtgaccgtgcccagcagcagatggcccagcgagaccttcacctgcaacgtggcccaccccgccaccaacaccaaggtggacaagcccgtggccaaggagtgcgagtgcaagtgcaactgcaacaactgcccctgccccggctgcggcctgctgggcggcnnnagcgtgttcatcttcccccccaagcccaaggacatcctggtgaccgccagaacccccaccgtgacctgcgtggtggtgnnnctggaccccgagaaccccgaggtgcagatcagctggttcgtggacagcaagcaggtgcagaccgccaacacccagcccagagaggagcagagcnnnnnnnnntacagagtggtgagcgtgctgcccatcggccaccaggactggctgagcggcaagcagttcaagtgcaaggtgaacaacaagnnnctgnnnagccccatcgaggagatcatcagcaagacccccggccaggcccaccagcccaacgtgtacgtgctgccccccagcagagacgagatgagcaagaacaccgtgaccctgacctgcctggtgaaggacttcttcccccccgagatcgacgtggagtggcagagcaacggccagcaggagcccgagagcaagtacagaatgacccccccccagctggacgaggacggcagctacttcctgtacagcaagctgagcgtggacaagagcagatggcagagaggcgacaccttcatctgcgccgtgatgcacgaggccctgcacaaccactacacccagatcagcctgagccacagccccggcaag

SEQ ID NO: 58 - protein, 448 aa, synthetic construct
  REGION 1..448: note = caninized mouse antibody
  VARIANT 237: note = misc_feature - Xaa can be any naturally occurring amino acid
  VARIANT 264: note = misc_feature - Xaa can be any naturally occurring amino acid
  VARIANT 296..298: note = misc_feature - Xaa can be any naturally occurring amino acid
  VARIANT 326: note = misc_feature - Xaa can be any naturally occurring amino acid
  VARIANT 328: note = misc_feature - Xaa can be any naturally occurring amino acid
EVQLVQSGAEVKKPGASVKVSCKASGYTFTTYGMSWVRQAPGKGLQWMGWINIYSGIPTYADDFKGRFALSLDTSTSTAYMELNSLRAEDTAVYYCARFDGPDYWGQGTLVTVSSASTTAPSVFPLAPSCGSQSGSTVALACLVSGYIPEPVTVSWNSVSLTSGVHTFPSVLQSSGLYSLSSMVTVPSSRWPSETFTCNVAHPATNTKVDKPVAKECECKCNCNNCPCPGCGLLGGXSVFIFPPKPKDILVTARTPTVTCVVVXLDPENPEVQISWFVDSKQVQTANTQPREEQSXXXYRVVSVLPIGHQDWLSGKQFKCKVNNKXLXSPIEEIISKTPGQAHQPNVYVLPPSRDEMSKNTVTLTCLVKDFFPPEIDVEWQSNGQQEPESKYRMTPPQLDEDGSYFLYSKLSVDKSRWQRGDTFICAVMHEALHNHYTQISLSHSPGK

SEQ ID NO: 59 - DNA, 1365 bp, synthetic construct
  misc_feature 1..1365: note = caninized mouse antibody
  misc_difference 730..732: note = n is a, c, g, or t
  misc_difference 811..813: note = n is a, c, g, or t
  misc_difference 907..915: note = n is a, c, g, or t
  misc_difference 997..999: note = n is a, c, g, or t
  misc_difference 1003..1005: note = n is a, c, g, or t
  source 1..1365: mol_type = other DNA
gaggtgcagctggtgcagagcgtggccgagctggtgaagcccggcgccagcgtgaaggtgagctgcaccgtgagcggcttcaacatcaagaacacctacatgcactgggtgagacaggcccccggcaagggcctgcagtggatcggcagaatcgaccccgccaacgtgaacaccaagtacgcccccaagttccagggcagagccaccatcaccgccgacaccagcaccaacaccgcctacatgcagctgagcagcctgagagccgaggacaccgccgtgtactactgcgccagaatctactacgactacgacggcgacatcgacgtgtggggccagggcaccctggtgaccgtgagcagcgccagcaccaccgcccccagcgtgttccccctggcccccagctgcggcagcaccagcggcagcaccgtggccctggcctgcctggtgagcggctacttccccgagcccgtgaccgtgagctggaacagcggcagcctgaccagcggcgtgcacaccttccccagcgtgctgcagagcagcggcctgtacagcctgagcagcatggtgaccgtgcccagcagcagatggcccagcgagaccttcacctgcaacgtggcccaccccgccagcaagaccaaggtggacaagcccgtgcccaagagagagaacggcagagtgcccagaccccccgactgccccaagtgccccgcccccgagatgctgggcggcnnnagcgtgttcatcttcccccccaagcccaaggacaccctgctgatcgccagaacccccgaggtgacctgcgtggtggtgnnnctggaccccgaggaccccgaggtgcagatcagctggttcgtggacggcaagcagatgcagaccgccaagacccagcccagagaggagcagttcnnnnnnnnntacagagtggtgagcgtgctgcccatcggccaccaggactggctgaagggcaagcagttcacctgcaaggtgaacaacaagnnnctgnnnagccccatcgagagaaccatcagcaaggccagaggccaggcccaccagcccagcgtgtacgtgctgccccccagcagagaggagctgagcaagaacaccgtgagcctgacctgcctgatcaaggacttcttcccccccgacatcgacgtggagtggcagagcaacggccagcaggagcccgagagcaagtacagaaccacccccccccagctggacgaggacggcagctacttcctgtacagcaagctgagcgtggacaagagcagatggcagagaggcgacaccttcatctgcgccgtgatgcacgaggccctgcacaaccactacacccaggagagcctgagccacagccccggcaag

SEQ ID NO: 60 - protein, 455 aa, synthetic construct
  REGION 1..455: note = caninized mouse antibody
  VARIANT 244: note = misc_feature - Xaa can be any naturally occurring amino acid
  VARIANT 271: note = misc_feature - Xaa can be any naturally occurring amino acid
  VARIANT 303..305: note = misc_feature - Xaa can be any naturally occurring amino acid
  VARIANT 333: note = misc_feature - Xaa can be any naturally occurring amino acid
  VARIANT 335: note = misc_feature - Xaa can be any naturally occurring amino acid
EVQLVQSVAELVKPGASVKVSCTVSGFNIKNTYMHWVRQAPGKGLQWIGRIDPANVNTKYAPKFQGRATITADTSTNTAYMQLSSLRAEDTAVYYCARIYYDYDGDIDVWGQGTLVTVSSASTTAPSVFPLAPSCGSTSGSTVALACLVSGYFPEPVTVSWNSGSLTSGVHTFPSVLQSSGLYSLSSMVTVPSSRWPSETFTCNVAHPASKTKVDKPVPKRENGRVPRPPDCPKCPAPEMLGGXSVFIFPPKPKDTLLIARTPEVTCVVVXLDPEDPEVQISWFVDGKQMQTAKTQPREEQFXXXYRVVSVLPIGHQDWLKGKQFTCKVNNKXLXSPIERTISKARGQAHQPSVYVLPPSREELSKNTVSLTCLIKDFFPPDIDVEWQSNGQQEPESKYRTTPPQLDEDGSYFLYSKLSVDKSRWQRGDTFICAVMHEALHNHYTQESLSHSPGK

SEQ ID NO: 61 - DNA, 1359 bp, synthetic construct
  misc_feature 1..1359: note = caninized mouse antibody
  misc_difference 724..726: note = n is a, c, g, or t
  misc_difference 805..807: note = n is a, c, g, or t
  misc_difference 901..909: note = n is a, c, g, or t
  misc_difference 991..993: note = n is a, c, g, or t
  misc_difference 997..999: note = n is a, c, g, or t
  source 1..1359: mol_type = other DNA
gaggtgcagctggtgcagagcgtggccgagctggtgaagcccggcgccagcgtgaaggtgagctgcaccgtgagcggcttcaacatcaagaacacctacatgcactgggtgagacaggcccccggcaagggcctgcagtggatcggcagaatcgaccccgccaacgtgaacaccaagtacgcccccaagttccagggcagagccaccatcaccgccgacaccagcaccaacaccgcctacatgcagctgagcagcctgagagccgaggacaccgccgtgtactactgcgccagaatctactacgactacgacggcgacatcgacgtgtggggccagggcaccctggtgaccgtgagcagcgccagcaccaccgcccccagcgtgttccccctggcccccagctgcggcagcaccagcggcagcaccgtggccctggcctgcctggtgagcggctacttccccgagcccgtgaccgtgagctggaacagcggcagcctgaccagcggcgtgcacaccttccccagcgtgctgcagagcagcggcctgtacagcctgagcagcatggtgaccgtgcccagcagcagatggcccagcgagaccttcacctgcaacgtggcccaccccgccagcaagaccaaggtggacaagcccgtggccaaggagtgcgagtgcaagtgcaactgcaacaactgcccctgccccggctgcggcctgctgggcggcnnnagcgtgttcatcttcccccccaagcccaaggacatcctggtgaccgccagaacccccaccgtgacctgcgtggtggtgnnnctggaccccgagaaccccgaggtgcagatcagctggttcgtggacagcaagcaggtgcagaccgccaacacccagcccagagaggagcagagcnnnnnnnnntacagagtggtgagcgtgctgcccatcggccaccaggactggctgagcggcaagcagttcaagtgcaaggtgaacaacaagnnnctgnnnagccccatcgaggagatcatcagcaagacccccggccaggcccaccagcccaacgtgtacgtgctgccccccagcagagacgagatgagcaagaacaccgtgaccctgacctgcctggtgaaggacttcttcccccccgagatcgacgtggagtggcagagcaacggccagcaggagcccgagagcaagtacagaatgacccccccccagctggacgaggacggcagctacttcctgtacagcaagctgagcgtggacaagagcagatggcagagaggcgacaccttcatctgcgccgtgatgcacgaggccctgcacaaccactacacccagatcagcctgagccacagccccggcaag

SEQ ID NO: 62 - protein, 453 aa, synthetic construct
  REGION 1..453: note = caninized mouse antibody
  VARIANT 242: note = misc_feature - Xaa can be any naturally occurring amino acid
  VARIANT 269: note = misc_feature - Xaa can be any naturally occurring amino acid
  VARIANT 301..303: note = misc_feature - Xaa can be any naturally occurring amino acid
  VARIANT 331: note = misc_feature - Xaa can be any naturally occurring amino acid
  VARIANT 333: note = misc_feature - Xaa can be any naturally occurring amino acid
EVQLVQSVAELVKPGASVKVSCTVSGFNIKNTYMHWVRQAPGKGLQWIGRIDPANVNTKYAPKFQGRATITADTSTNTAYMQLSSLRAEDTAVYYCARIYYDYDGDIDVWGQGTLVTVSSASTTAPSVFPLAPSCGSTSGSTVALACLVSGYFPEPVTVSWNSGSLTSGVHTFPSVLQSSGLYSLSSMVTVPSSRWPSETFTCNVAHPASKTKVDKPVAKECECKCNCNNCPCPGCGLLGGXSVFIFPPKPKDILVTARTPTVTCVVVXLDPENPEVQISWFVDSKQVQTANTQPREEQSXXXYRVVSVLPIGHQDWLSGKQFKCKVNNKXLXSPIEEIISKTPGQAHQPNVYVLPPSRDEMSKNTVTLTCLVKDFFPPEIDVEWQSNGQQEPESKYRMTPPQLDEDGSYFLYSKLSVDKSRWQRGDTFICAVMHEALHNHYTQISLSHSPGK

SEQ ID NO: 63 - DNA, 1350 bp, synthetic construct
  misc_feature 1..1350: note = caninized mouse antibody
  misc_difference 715..717: note = n is a, c, g, or t
  misc_difference 796..798: note = n is a, c, g, or t
  misc_difference 892..900: note = n is a, c, g, or t
  misc_difference 982..984: note = n is a, c, g, or t
  misc_difference 988..990: note = n is a, c, g, or t
  source 1..1350: mol_type = other DNA
gaggtgcagctggtgcagagcggcgccgaggtgaagaagcccggcgccagcgtgaaggtgagctgcaaggccagcggctacaccttcaccacctacggcatgagctgggtgagacaggcccccggcaagggcctgcagtggatgggctggatcaacatctacagcggcatgcccacctacgccgacgacttcaagggcagattcgccctgagcctggacaccagcaccagcaccgcctacatggagctgaacagcctgagagccgaggacaccgccgtgtactactgcaccagattcgacggccccgactactggggccagggcaccctggtgaccgtgagcagcgccagcaccaccgcccccagcgtgttccccctggcccccagctgcggcagcaccagcggcagcaccgtggccctggcctgcctggtgagcggctacttccccgagcccgtgaccgtgagctggaacagcggcagcctgaccagcggcgtgcacaccttccccagcgtgctgcagagcagcggcctgtacagcctgagcagcatggtgaccgtgcccagcagcagatggcccagcgagaccttcacctgcaacgtggcccaccccgccagcaagaccaaggtggacaagcccgtgcccaagagagagaacggcagagtgcccagaccccccgactgccccaagtgccccgcccccgagatgctgggcggcnnnagcgtgttcatcttcccccccaagcccaaggacaccctgctgatcgccagaacccccgaggtgacctgcgtggtggtgnnnctggaccccgaggaccccgaggtgcagatcagctggttcgtggacggcaagcagatgcagaccgccaagacccagcccagagaggagcagttcnnnnnnnnntacagagtggtgagcgtgctgcccatcggccaccaggactggctgaagggcaagcagttcacctgcaaggtgaacaacaagnnnctgnnnagccccatcgagagaaccatcagcaaggccagaggccaggcccaccagcccagcgtgtacgtgctgccccccagcagagaggagctgagcaagaacaccgtgagcctgacctgcctgatcaaggacttcttcccccccgacatcgacgtggagtggcagagcaacggccagcaggagcccgagagcaagtacagaaccacccccccccagctggacgaggacggcagctacttcctgtacagcaagctgagcgtggacaagagcagatggcagagaggcgacaccttcatctgcgccgtgatgcacgaggccctgcacaaccactacacccaggagagcctgagccacagccccggcaag

SEQ ID NO: 64 - protein, 450 aa, synthetic construct
  REGION 1..450: note = caninized mouse antibody
  VARIANT 239: note = misc_feature - Xaa can be any naturally occurring amino acid
  VARIANT 266: note = misc_feature - Xaa can be any naturally occurring amino acid
  VARIANT 298..300: note = misc_feature - Xaa can be any naturally occurring amino acid
  VARIANT 328: note = misc_feature - Xaa can be any naturally occurring amino acid
  VARIANT 330: note = misc_feature - Xaa can be any naturally occurring amino acid
EVQLVQSGAEVKKPGASVKVSCKASGYTFTTYGMSWVRQAPGKGLQWMGWINIYSGMPTYADDFKGRFALSLDTSTSTAYMELNSLRAEDTAVYYCTRFDGPDYWGQGTLVTVSSASTTAPSVFPLAPSCGSTSGSTVALACLVSGYFPEPVTVSWNSGSLTSGVHTFPSVLQSSGLYSLSSMVTVPSSRWPSETFTCNVAHPASKTKVDKPVPKRENGRVPRPPDCPKCPAPEMLGGXSVFIFPPKPKDTLLIARTPEVTCVVVXLDPEDPEVQISWFVDGKQMQTAKTQPREEQFXXXYRVVSVLPIGHQDWLKGKQFTCKVNNKXLXSPIERTISKARGQAHQPSVYVLPPSREELSKNTVSLTCLIKDFFPPDIDVEWQSNGQQEPESKYRTTPPQLDEDGSYFLYSKLSVDKSRWQRGDTFICAVMHEALHNHYTQESLSHSPGK

SEQ ID NO: 65 - DNA, 1344 bp, synthetic construct
  misc_feature 1..1344: note = caninized mouse antibody
  misc_difference 709..711: note = n is a, c, g, or t
  misc_difference 790..792: note = n is a, c, g, or t
  misc_difference 886..894: note = n is a, c, g, or t
  misc_difference 976..978: note = n is a, c, g, or t
  misc_difference 982..984: note = n is a, c, g, or t
  source 1..1344: mol_type = other DNA
gaggtgcagctggtgcagagcggcgccgaggtgaagaagcccggcgccagcgtgaaggtgagctgcaaggccagcggctacaccttcaccacctacggcatgagctgggtgagacaggcccccggcaagggcctgcagtggatgggctggatcaacatctacagcggcatgcccacctacgccgacgacttcaagggcagattcgccctgagcctggacaccagcaccagcaccgcctacatggagctgaacagcctgagagccgaggacaccgccgtgtactactgcaccagattcgacggccccgactactggggccagggcaccctggtgaccgtgagcagcgccagcaccaccgcccccagcgtgttccccctggcccccagctgcggcagcaccagcggcagcaccgtggccctggcctgcctggtgagcggctacttccccgagcccgtgaccgtgagctggaacagcggcagcctgaccagcggcgtgcacaccttccccagcgtgctgcagagcagcggcctgtacagcctgagcagcatggtgaccgtgcccagcagcagatggcccagcgagaccttcacctgcaacgtggcccaccccgccagcaagaccaaggtggacaagcccgtggccaaggagtgcgagtgcaagtgcaactgcaacaactgcccctgccccggctgcggcctgctgggcggcnnnagcgtgttcatcttcccccccaagcccaaggacatcctggtgaccgccagaacccccaccgtgacctgcgtggtggtgnnnctggaccccgagaaccccgaggtgcagatcagctggttcgtggacagcaagcaggtgcagaccgccaacacccagcccagagaggagcagagcnnnnnnnnntacagagtggtgagcgtgctgcccatcggccaccaggactggctgagcggcaagcagttcaagtgcaaggtgaacaacaagnnnctgnnnagccccatcgaggagatcatcagcaagacccccggccaggcccaccagcccaacgtgtacgtgctgccccccagcagagacgagatgagcaagaacaccgtgaccctgacctgcctggtgaaggacttcttcccccccgagatcgacgtggagtggcagagcaacggccagcaggagcccgagagcaagtacagaatgacccccccccagctggacgaggacggcagctacttcctgtacagcaagctgagcgtggacaagagcagatggcagagaggcgacaccttcatctgcgccgtgatgcacgaggccctgcacaaccactacacccagatcagcctgagccacagccccggcaag

SEQ ID NO: 66 - protein, 448 aa, synthetic construct
  REGION 1..448: note = caninized mouse antibody
  VARIANT 237: note = misc_feature - Xaa can be any naturally occurring amino acid
  VARIANT 264: note = misc_feature - Xaa can be any naturally occurring amino acid
  VARIANT 296..298: note = misc_feature - Xaa can be any naturally occurring amino acid
  VARIANT 326: note = misc_feature - Xaa can be any naturally occurring amino acid
  VARIANT 328: note = misc_feature - Xaa can be any naturally occurring amino acid
EVQLVQSGAEVKKPGASVKVSCKASGYTFTTYGMSWVRQAPGKGLQWMGWINIYSGMPTYADDFKGRFALSLDTSTSTAYMELNSLRAEDTAVYYCTRFDGPDYWGQGTLVTVSSASTTAPSVFPLAPSCGSTSGSTVALACLVSGYFPEPVTVSWNSGSLTSGVHTFPSVLQSSGLYSLSSMVTVPSSRWPSETFTCNVAHPASKTKVDKPVAKECECKCNCNNCPCPGCGLLGGXSVFIFPPKPKDILVTARTPTVTCVVVXLDPENPEVQISWFVDSKQVQTANTQPREEQSXXXYRVVSVLPIGHQDWLSGKQFKCKVNNKXLXSPIEEIISKTPGQAHQPNVYVLPPSRDEMSKNTVTLTCLVKDFFPPEIDVEWQSNGQQEPESKYRMTPPQLDEDGSYFLYSKLSVDKSRWQRGDTFICAVMHEALHNHYTQISLSHSPGK

SEQ ID NO: 67 - DNA, 1338 bp, synthetic construct
  misc_feature 1..1338: note = caninized mouse antibody
  source 1..1338: mol_type = other DNA
gaggtgcagctggtgcagagcggcggcgacctggtgaagcccggcggcagcgtgagactgagctgcgtggccagcggctacaccttcaccacctacggcatgagctgggtgagacaggcccccggcaagggcctgcagtggatgggctggatcaacatctacagcggcatccccacctacgccgacgacttcaagggcagattcaccttcagcctggacaccgccaagaacaccgcctacctgcagctgaacagcctgagagccgaggacaccgccgtgtactactgcaccagattcgacggccccgactactggggccagggcaccctggtgaccgtgagcagcgccagcaccaccgcccccagcgtgttccccctggcccccagctgcggcagcaccagcggcagcaccgtggccctggcctgcctggtgagcggctacttccccgagcccgtgaccgtgagctggaacagcggcagcctgaccagcggcgtgcacaccttccccagcgtgctgcagagcagcggcctgcacagcctgagcagcatggtgaccgtgcccagcagcagatggcccagcgagaccttcacctgcaacgtggtgcaccccgccagcaacaccaaggtggacaagcccgtgttcaacgagtgcagatgcaccgacacccccccctgccccgtgcccgagcccctgggcggccccagcgtgctgatcttcccccccaagcccaaggacatcctgagaatcaccagaacccccgaggtgacctgcgtggtgctggacctgggcagagaggaccccgaggtgcagatcagctggttcgtggacggcaaggaggtgcacaccgccaagacccagagcagagagcagcagttcaacggcacctacagagtggtgagcgtgctgcccatcgagcaccaggactggctgaccggcaaggagttcaagtgcagagtgaaccacatcgacctgcccagccccatcgagagaaccatcagcaaggccagaggcagagcccacaagcccagcgtgtacgtgctgccccccagccccaaggagctgagcagcagcgacaccgtgagcatcacctgcctgatcaaggacttctacccccccgacatcgacgtggagtggcagagcaacggccagcaggagcccgagagaaagcacagaatgacccccccccagctggacgaggacggcagctacttcctgtacagcaagctgagcgtggacaagagcagatggcagcagggcgaccccttcacctgcgccgtgatgcacgagaccctgcagaaccactacaccgacctgagcctgagccacagccccggcaag

SEQ ID NO: 68 - protein, 446 aa, synthetic construct
  REGION 1..446: note = caninized mouse antibody
EVQLVQSGGDLVKPGGSVRLSCVASGYTFTTYGMSWVRQAPGKGLQWMGWINIYSGIPTYADDFKGRFTFSLDTAKNTAYLQLNSLRAEDTAVYYCTRFDGPDYWGQGTLVTVSSASTTAPSVFPLAPSCGSTSGSTVALACLVSGYFPEPVTVSWNSGSLTSGVHTFPSVLQSSGLHSLSSMVTVPSSRWPSETFTCNVVHPASNTKVDKPVFNECRCTDTPPCPVPEPLGGPSVLIFPPKPKDILRITRTPEVTCVVLDLGREDPEVQISWFVDGKEVHTAKTQSREQQFNGTYRVVSVLPIEHQDWLTGKEFKCRVNHIDLPSPIERTISKARGRAHKPSVYVLPPSPKELSSSDTVSITCLIKDFYPPDIDVEWQSNGQQEPERKHRMTPPQLDEDGSYFLYSKLSVDKSRWQQGDPFTCAVMHETLQNHYTDLSLSHSPGK

SEQ ID NO: 69 - DNA, 1338 bp, synthetic construct
  misc_feature 1..1338: note = caninized mouse antibody
  source 1..1338: mol_type = other DNA
gaggtgcagctggtgcagagcggcggcgacctggtgaagcccggcggcagcgtgagactgagctgcgtggccagcggctacaccttcaccacctacggcatgagctgggtgagacaggcccccggcaagggcctgcagtggatgggctggatcaacatctacagcggcatccccacctacgccgacgacttcaagggcagattcaccttcagcctggacaccgccaagaacaccgcctacctgcagctgaacagcctgagagccgaggacaccgccgtgtactactgcaccagattcgacggccccgactactggggccagggcaccctggtgaccgtgagcagcgccagcaccaccgcccccagcgtgttccccctggcccccagctgcggcagcaccagcggcagcaccgtggccctggcctgcctggtgagcggctacttccccgagcccgtgaccgtgagctggaacagcggcagcctgaccagcggcgtgcacaccttccccagcgtgctgcagagcagcggcctgtacagcctgagcagcaccgtgaccgtgcccagcagcagatggcccagcgagaccttcacctgcaacgtggtgcaccccgccagcaacaccaaggtggacaagcccgtgcccaaggagagcacctgcaagtgcatcagcccctgccccgtgcccgagagcctgggcggccccagcgtgttcatcttcccccccaagcccaaggacatcctgagaatcaccagaacccccgagatcacctgcgtggtgctggacctgggcagagaggaccccgaggtgcagatcagctggttcgtggacggcaaggaggtgcacaccgccaagacccagcccagagagcagcagttcaacagcacctacagagtggtgagcgtgctgcccatcgagcaccaggactggctgaccggcaaggagttcaagtgcagagtgaaccacatcggcctgcccagccccatcgagagaaccatcagcaaggccagaggccaggcccaccagcccagcgtgtacgtgctgccccccagccccaaggagctgagcagcagcgacaccgtgaccctgacctgcctgatcaaggacttcttcccccccgagatcgacgtggagtggcagagcaacggccagcccgagcccgagagcaagtaccacaccaccgccccccagctggacgaggacggcagctacttcctgtacagcaagctgagcgtggacaagagcagatggcagcagggcgacaccttcacctgcgccgtgatgcacgaggccctgcagaaccactacaccgacctgagcctgagccacagccccggcaag

SEQ ID NO: 70 - protein, 446 aa, synthetic construct
  REGION 1..446: note = caninized mouse antibody
EVQLVQSGGDLVKPGGSVRLSCVASGYTFTTYGMSWVRQAPGKGLQWMGWINIYSGIPTYADDFKGRFTFSLDTAKNTAYLQLNSLRAEDTAVYYCTRFDGPDYWGQGTLVTVSSASTTAPSVFPLAPSCGSTSGSTVALACLVSGYFPEPVTVSWNSGSLTSGVHTFPSVLQSSGLYSLSSTVTVPSSRWPSETFTCNVVHPASNTKVDKPVPKESTCKCISPCPVPESLGGPSVFIFPPKPKDILRITRTPEITCVVLDLGREDPEVQISWFVDGKEVHTAKTQPREQQFNSTYRVVSVLPIEHQDWLTGKEFKCRVNHIGLPSPIERTISKARGQAHQPSVYVLPPSPKELSSSDTVTLTCLIKDFFPPEIDVEWQSNGQPEPESKYHTTAPQLDEDGSYFLYSKLSVDKSRWQQGDTFTCAVMHEALQNHYTDLSLSHSPGK

SEQ ID NO: 71 - DNA, 672 bp, synthetic construct
  misc_feature 1..672: note = caninized mouse antibody
  source 1..672: mol_type = other DNA
gacatcgtgatgacccagacccccctgagcctgagcgtgagccccggcgagcccgccagcatgagctgcaagagcagccagagcctgctgaacagcgtgaaccagaagaactacctggcctggtacagacagaagcccggccagagcccccaggtgctggtgtacttcgccagcgccagagtgagcggcgtgcccgacagattcatcggcagcggcagcggcaccgacttcaccctgagaatcagcagagtggaggccgacgacctgggcgtgtactactgccagcagtacttcagcacccccctgaccttcggccagggcaccaagctggagctgaagagaaacgacgcccagcccgccgtgtacctgttccagcccagccccgaccagctgcacaccggcagcgccagcgtggtgtgcctgctgaacagcttctaccccaaggacatcaacgtgaagtggaaggtggacggcgtgatccaggacaccggcatccaggagagcgtgaccgagcaggacagcaaggacagcacctacagcctgagcagcaccctgaccatgagcagcaccgagtacctgagccacgagctgtacagctgcgagatcacccacaagagcctgcccagcaccctgatcaagagcttccagagaagcgagtgccagagagtggac

SEQ ID NO: 72 - protein, 224 aa, synthetic construct
  REGION 1..224: note = caninized mouse antibody
DIVMTQTPLSLSVSPGEPASMSCKSSQSLLNSVNQKNYLAWYRQKPGQSPQVLVYFASARVSGVPDRFIGSGSGTDFTLRISRVEADDLGVYYCQQYFSTPLTFGQGTKLELKRNDAQPAVYLFQPSPDQLHTGSASVVCLLNSFYPKDINVKWKVDGVIQDTGIQESVTEQDSKDSTYSLSSTLTMSSTEYLSHELYSCEITHKSLPSTLIKSFQRSECQRVD

SEQ ID NO: 73 - DNA, 1353 bp, synthetic construct
  misc_feature 1..1353: note = caninized mouse antibody
  source 1..1353: mol_type = other DNA
gaggtgcagctggtgcagagcggcggcgacctggtgaagcccggcggcagcgtgagactgagctgcgtggccagcggcttcaacatcaagaacacctacatgcactgggtgagacaggcccccggcaagggcctgcagtggatcggcagaatcgcccccgccaacgtggacaccaagtacgcccccaagttccagggcaaggccaccatcagcgccgacaccgccaagaacaccgcctacatgcagctgaacagcctgagagccgaggacaccgccgtgtactactgcgtgctgatctactacgactacgacggcgacatcgacgtgtggggccagggcaccctggtgaccgtgagcagcgccagcaccaccgcccccagcgtgttccccctggcccccagctgcggcagcaccagcggcagcaccgtggccctggcctgcctggtgagcggctacttccccgagcccgtgaccgtgagctggaacagcggcagcctgaccagcggcgtgcacaccttccccagcgtgctgcagagcagcggcctgcacagcctgagcagcatggtgaccgtgcccagcagcagatggcccagcgagaccttcacctgcaacgtggtgcaccccgccagcaacaccaaggtggacaagcccgtgttcaacgagtgcagatgcaccgacacccccccctgccccgtgcccgagcccctgggcggccccagcgtgctgatcttcccccccaagcccaaggacatcctgagaatcaccagaacccccgaggtgacctgcgtggtgctggacctgggcagagaggaccccgaggtgcagatcagctggttcgtggacggcaaggaggtgcacaccgccaagacccagagcagagagcagcagttcaacggcacctacagagtggtgagcgtgctgcccatcgagcaccaggactggctgaccggcaaggagttcaagtgcagagtgaaccacatcgacctgcccagccccatcgagagaaccatcagcaaggccagaggcagagcccacaagcccagcgtgtacgtgctgccccccagccccaaggagctgagcagcagcgacaccgtgagcatcacctgcctgatcaaggacttctacccccccgacatcgacgtggagtggcagagcaacggccagcaggagcccgagagaaagcacagaatgacccccccccagctggacgaggacggcagctacttcctgtacagcaagctgagcgtggacaagagcagatggcagcagggcgaccccttcacctgcgccgtgatgcacgagaccctgcagaaccactacaccgacctgagcctgagccacagccccggcaag

SEQ ID NO: 74 - protein, 451 aa, synthetic construct
  REGION 1..451: note = caninized mouse antibody
EVQLVQSGGDLVKPGGSVRLSCVASGFNIKNTYMHWVRQAPGKGLQWIGRIAPANVDTKYAPKFQGKATISADTAKNTAYMQLNSLRAEDTAVYYCVLIYYDYDGDIDVWGQGTLVTVSSASTTAPSVFPLAPSCGSTSGSTVALACLVSGYFPEPVTVSWNSGSLTSGVHTFPSVLQSSGLHSLSSMVTVPSSRWPSETFTCNVVHPASNTKVDKPVFNECRCTDTPPCPVPEPLGGPSVLIFPPKPKDILRITRTPEVTCVVLDLGREDPEVQISWFVDGKEVHTAKTQSREQQFNGTYRVVSVLPIEHQDWLTGKEFKCRVNHIDLPSPIERTISKARGRAHKPSVYVLPPSPKELSSSDTVSITCLIKDFYPPDIDVEWQSNGQQEPERKHRMTPPQLDEDGSYFLYSKLSVDKSRWQQGDPFTCAVMHETLQNHYTDLSLSHSPGK

SEQ ID NO: 75 - DNA, 1353 bp, synthetic construct
  misc_feature 1..1353: note = caninized mouse antibody
  source 1..1353: mol_type = other DNA
gaggtgcagctggtgcagagcggcggcgacctggtgaagcccggcggcagcgtgagactgagctgcgtggccagcggcttcaacatcaagaacacctacatgcactgggtgagacaggcccccggcaagggcctgcagtggatcggcagaatcgcccccgccaacgtggacaccaagtacgcccccaagttccagggcaaggccaccatcagcgccgacaccgccaagaacaccgcctacatgcagctgaacagcctgagagccgaggacaccgccgtgtactactgcgtgctgatctactacgactacgacggcgacatcgacgtgtggggccagggcaccctggtgaccgtgagcagcgccagcaccaccgcccccagcgtgttccccctggcccccagctgcggcagcaccagcggcagcaccgtggccctggcctgcctggtgagcggctacttccccgagcccgtgaccgtgagctggaacagcggcagcctgaccagcggcgtgcacaccttccccagcgtgctgcagagcagcggcctgtacagcctgagcagcaccgtgaccgtgcccagcagcagatggcccagcgagaccttcacctgcaacgtggtgcaccccgccagcaacaccaaggtggacaagcccgtgcccaaggagagcacctgcaagtgcatcagcccctgccccgtgcccgagagcctgggcggccccagcgtgttcatcttcccccccaagcccaaggacatcctgagaatcaccagaacccccgagatcacctgcgtggtgctggacctgggcagagaggaccccgaggtgcagatcagctggttcgtggacggcaaggaggtgcacaccgccaagacccagcccagagagcagcagttcaacagcacctacagagtggtgagcgtgctgcccatcgagcaccaggactggctgaccggcaaggagttcaagtgcagagtgaaccacatcggcctgcccagccccatcgagagaaccatcagcaaggccagaggccaggcccaccagcccagcgtgtacgtgctgccccccagccccaaggagctgagcagcagcgacaccgtgaccctgacctgcctgatcaaggacttcttcccccccgagatcgacgtggagtggcagagcaacggccagcccgagcccgagagcaagtaccacaccaccgccccccagctggacgaggacggcagctacttcctgtacagcaagctgagcgtggacaagagcagatggcagcagggcgacaccttcacctgcgccgtgatgcacgaggccctgcagaaccactacaccgacctgagcctgagccacagccccggcaag

SEQ ID NO: 76 - protein, 451 aa, synthetic construct
  REGION 1..451: note = caninized mouse antibody
EVQLVQSGGDLVKPGGSVRLSCVASGFNIKNTYMHWVRQAPGKGLQWIGRIAPANVDTKYAPKFQGKATISADTAKNTAYMQLNSLRAEDTAVYYCVLIYYDYDGDIDVWGQGTLVTVSSASTTAPSVFPLAPSCGSTSGSTVALACLVSGYFPEPVTVSWNSGSLTSGVHTFPSVLQSSGLYSLSSTVTVPSSRWPSETFTCNVVHPASNTKVDKPVPKESTCKCISPCPVPESLGGPSVFIFPPKPKDILRITRTPEITCVVLDLGREDPEVQISWFVDGKEVHTAKTQPREQQFNSTYRVVSVLPIEHQDWLTGKEFKCRVNHIGLPSPIERTISKARGQAHQPSVYVLPPSPKELSSSDTVTLTCLIKDFFPPEIDVEWQSNGQPEPESKYHTTAPQLDEDGSYFLYSKLSVDKSRWQQGDTFTCAVMHEALQNHYTDLSLSHSPGK

SEQ ID NO: 77 - DNA, 654 bp, synthetic construct
  misc_feature 1..654: note = caninized mouse antibody
  source 1..654: mol_type = other DNA
gacatcgtgatgacccagacccccctgagcctgagcgtgagcctgggcgagcccgccagcatcagctgccacgccagccagaacatcaacgtgtggctgagctggtacagacagaagcccggccagatcccccagctgctgatctacaaggccagccacctgcacaccggcgtgcccgacagattcagcggcagcggcagcggcaccgacttcaccctgagaatcagcagagtggaggccgacgacgccggcgtgtactactgccagcagggccagagctggcccctgaccttcggccagggcaccaaggtggagatcaagagaaacgacgcccagcccgccgtgtacctgttccagcccagccccgaccagctgcacaccggcagcgccagcgtggtgtgcctgctgaacagcttctaccccaaggacatcaacgtgaagtggaaggtggacggcgtgatccaggacaccggcatccaggagagcgtgaccgagcaggacagcaaggacagcacctacagcctgagcagcaccctgaccatgagcagcaccgagtacctgagccacgagctgtacagctgcgagatcacccacaagagcctgcccagcaccctgatcaagagcttccagagaagcgagtgccagagagtggac

SEQ ID NO: 78 - protein, 218 aa, synthetic construct
  REGION 1..218: note = caninized mouse antibody
DIVMTQTPLSLSVSLGEPASISCHASQNINVWLSWYRQKPGQIPQLLIYKASHLHTGVPDRFSGSGSGTDFTLRISRVEADDAGVYYCQQGQSWPLTFGQGTKVEIKRNDAQPAVYLFQPSPDQLHTGSASVVCLLNSFYPKDINVKWKVDGVIQDTGIQESVTEQDSKDSTYSLSSTLTMSSTEYLSHELYSCEITHKSLPSTLIKSFQRSECQRVD

SEQ ID NO: 79 - DNA, 1359 bp, synthetic construct
  misc_feature 1..1359: note = caninized mouse antibody
  source 1..1359: mol_type = other DNA
gaggtgcagctggtgcagagcggcggcgacctggtgaagcccggcggcagcgtgagactgagctgcgtggccagcggctacaccttcaccagatacaacatgcactgggtgagacaggcccccggcaagggcctgcagtggatcggcaccatctaccccggctacggcgacaccagctacaaccagaagttcaagggcaaggccaccctgagcgtggacatcgccaagaacaccgcctacatgcagctgaacagcctgagagccgaggacaccgccgtgtacttctgcagcagagagttcgccgacgactaccccatcccccccttcgactactggggccagggcaccctggtgaccgtgagcagcgccagcaccaccgcccccagcgtgttccccctggcccccagctgcggcagcaccagcggcagcaccgtggccctggcctgcctggtgagcggctacttccccgagcccgtgaccgtgagctggaacagcggcagcctgaccagcggcgtgcacaccttccccagcgtgctgcagagcagcggcctgcacagcctgagcagcatggtgaccgtgcccagcagcagatggcccagcgagaccttcacctgcaacgtggtgcaccccgccagcaacaccaaggtggacaagcccgtgttcaacgagtgcagatgcaccgacacccccccctgccccgtgcccgagcccctgggcggccccagcgtgctgatcttcccccccaagcccaaggacatcctgagaatcaccagaacccccgaggtgacctgcgtggtgctggacctgggcagagaggaccccgaggtgcagatcagctggttcgtggacggcaaggaggtgcacaccgccaagacccagagcagagagcagcagttcaacggcacctacagagtggtgagcgtgctgcccatcgagcaccaggactggctgaccggcaaggagttcaagtgcagagtgaaccacatcgacctgcccagccccatcgagagaaccatcagcaaggccagaggcagagcccacaagcccagcgtgtacgtgctgccccccagccccaaggagctgagcagcagcgacaccgtgagcatcacctgcctgatcaaggacttctacccccccgacatcgacgtggagtggcagagcaacggccagcaggagcccgagagaaagcacagaatgacccccccccagctggacgaggacggcagctacttcctgtacagcaagctgagcgtggacaagagcagatggcagcagggcgaccccttcacctgcgccgtgatgcacgagaccctgcagaaccactacaccgacctgagcctgagccacagccccggcaag

SEQ ID NO: 80 - protein, 453 aa, synthetic construct
  REGION 1..453: note = caninized mouse antibody
EVQLVQSGGDLVKPGGSVRLSCVASGYTFTRYNMHWVRQAPGKGLQWIGTIYPGYGDTSYNQKFKGKATLSVDIAKNTAYMQLNSLRAEDTAVYFCSREFADDYPIPPFDYWGQGTLVTVSSASTTAPSVFPLAPSCGSTSGSTVALACLVSGYFPEPVTVSWNSGSLTSGVHTFPSVLQSSGLHSLSSMVTVPSSRWPSETFTCNVVHPASNTKVDKPVFNECRCTDTPPCPVPEPLGGPSVLIFPPKPKDILRITRTPEVTCVVLDLGREDPEVQISWFVDGKEVHTAKTQSREQQFNGTYRVVSVLPIEHQDWLTGKEFKCRVNHIDLPSPIERTISKARGRAHKPSVYVLPPSPKELSSSDTVSITCLIKDFYPPDIDVEWQSNGQQEPERKHRMTPPQLDEDGSYFLYSKLSVDKSRWQQGDPFTCAVMHETLQNHYTDLSLSHSPGK

SEQ ID NO: 81 - DNA, 1359 bp, synthetic construct
  misc_feature 1..1359: note = caninized mouse antibody
  source 1..1359: mol_type = other DNA
gaggtgcagctggtgcagagcggcggcgacctggtgaagcccggcggcagcgtgagactgagctgcgtggccagcggctacaccttcaccagatacaacatgcactgggtgagacaggcccccggcaagggcctgcagtggatcggcaccatctaccccggctacggcgacaccagctacaaccagaagttcaagggcaaggccaccctgagcgtggacatcgccaagaacaccgcctacatgcagctgaacagcctgagagccgaggacaccgccgtgtacttctgcagcagagagttcgccgacgactaccccatcccccccttcgactactggggccagggcaccctggtgaccgtgagcagcgccagcaccaccgcccccagcgtgttccccctggcccccagctgcggcagcaccagcggcagcaccgtggccctggcctgcctggtgagcggctacttccccgagcccgtgaccgtgagctggaacagcggcagcctgaccagcggcgtgcacaccttccccagcgtgctgcagagcagcggcctgtacagcctgagcagcaccgtgaccgtgcccagcagcagatggcccagcgagaccttcacctgcaacgtggtgcaccccgccagcaacaccaaggtggacaagcccgtgcccaaggagagcacctgcaagtgcatcagcccctgccccgtgcccgagagcctgggcggccccagcgtgttcatcttcccccccaagcccaaggacatcctgagaatcaccagaacccccgagatcacctgcgtggtgctggacctgggcagagaggaccccgaggtgcagatcagctggttcgtggacggcaaggaggtgcacaccgccaagacccagcccagagagcagcagttcaacagcacctacagagtggtgagcgtgctgcccatcgagcaccaggactggctgaccggcaaggagttcaagtgcagagtgaaccacatcggcctgcccagccccatcgagagaaccatcagcaaggccagaggccaggcccaccagcccagcgtgtacgtgctgccccccagccccaaggagctgagcagcagcgacaccgtgaccctgacctgcctgatcaaggacttcttcccccccgagatcgacgtggagtggcagagcaacggccagcccgagcccgagagcaagtaccacaccaccgccccccagctggacgaggacggcagctacttcctgtacagcaagctgagcgtggacaagagcagatggcagcagggcgacaccttcacctgcgccgtgatgcacgaggccctgcagaaccactacaccgacctgagcctgagccacagccccggcaag

SEQ ID NO: 82 - protein, 453 aa, synthetic construct
  REGION 1..453: note = caninized mouse antibody
EVQLVQSGGDLVKPGGSVRLSCVASGYTFTRYNMHWVRQAPGKGLQWIGTIYPGYGDTSYNQKFKGKATLSVDIAKNTAYMQLNSLRAEDTAVYFCSREFADDYPIPPFDYWGQGTLVTVSSASTTAPSVFPLAPSCGSTSGSTVALACLVSGYFPEPVTVSWNSGSLTSGVHTFPSVLQSSGLYSLSSTVTVPSSRWPSETFTCNVVHPASNTKVDKPVPKESTCKCISPCPVPESLGGPSVFIFPPKPKDILRITRTPEITCVVLDLGREDPEVQISWFVDGKEVHTAKTQPREQQFNSTYRVVSVLPIEHQDWLTGKEFKCRVNHIGLPSPIERTISKARGQAHQPSVYVLPPSPKELSSSDTVTLTCLIKDFFPPEIDVEWQSNGQPEPESKYHTTAPQLDEDGSYFLYSKLSVDKSRWQQGDTFTCAVMHEALQNHYTDLSLSHSPGK

SEQ ID NO: 83 - DNA, 666 bp, synthetic construct
  misc_feature 1..666: note = caninized mouse antibody
  source 1..666: mol_type = other DNA
gacatcgtgatgacccagacccccctgagcctgcccgtgagcctgggcgagcccgccagcatcagctgcagaagcagccagaacatcgtgcacagcaacggcaacacctacctggagtggtacagacagaagcccggccagagcccccagctgctgatctacaaggtgagcaacagattcagcggcgtgcccgacagattcagcggcagcggcagcggcaccgacttcaccctgagaatcagcagagtggaggccgacgacgccggcgtgtactactgcttccagggcagccacgtgccctacaccttcggccagggcaccaaggtggagatcaagagagacgcccagcccgccgtgtacctgttccagcccagccccgaccagctgcacaccggcagcgccagcgtggtgtgcctgctgaacagcttctaccccaaggacatcaacgtgaagtggaaggtggacggcgtgatccaggacaccggcatccaggagagcgtgaccgagcaggacagcaaggacagcacctacagcctgagcagcaccctgaccatgagcagcaccgagtacctgagccacgagctgtacagctgcgagatcacccacaagagcctgcccagcaccctgatcaagagcttccagagaagcgagtgccagagagtggac

SEQ ID NO: 84 - protein, 222 aa, synthetic construct
  REGION 1..222: note = caninized mouse antibody
DIVMTQTPLSLPVSLGEPASISCRSSQNIVHSNGNTYLEWYRQKPGQSPQLLIYKVSNRFSGVPDRFSGSGSGTDFTLRISRVEADDAGVYYCFQGSHVPYTFGQGTKVEIKRDAQPAVYLFQPSPDQLHTGSASVVCLLNSFYPKDINVKWKVDGVIQDTGIQESVTEQDSKDSTYSLSSTLTMSSTEYLSHELYSCEITHKSLPSTLIKSFQRSECQRVD

SEQ ID NO: 85 - DNA, 1338 bp, synthetic construct
  misc_feature 1..1338: note = caninized mouse antibody
  source 1..1338: mol_type = other DNA
gaggtgcagctggtgcagagcggccccggcctggtgaagcccagccagagcctgagcctgacctgcgtggtgagcggcttcagcctgaccagctacggcgtgcactgggtgagacaggcccccggcaagggcctgcagtggatgggctggatcaacatctacagcggcatccccacctacgccgacgacttcaagggcagattcaccttcagcctggacaccgccaagaacaccgcctacctgcagctgagcagcctgagagccgaggacaccgccgtgtactactgcgccagattcgacggccccgactactggggccagggcaccctggtgaccgtgagcagcgccagcaccaccgcccccagcgtgttccccctggcccccagctgcggcagcaccagcggcagcaccgtggccctggcctgcctggtgagcggctacttccccgagcccgtgaccgtgagctggaacagcggcagcctgaccagcggcgtgcacaccttccccagcgtgctgcagagcagcggcctgcacagcctgagcagcatggtgaccgtgcccagcagcagatggcccagcgagaccttcacctgcaacgtggtgcaccccgccagcaacaccaaggtggacaagcccgtgttcaacgagtgcagatgcaccgacacccccccctgccccgtgcccgagcccctgggcggccccagcgtgctgatcttcccccccaagcccaaggacatcctgagaatcaccagaacccccgaggtgacctgcgtggtgctggacctgggcagagaggaccccgaggtgcagatcagctggttcgtggacggcaaggaggtgcacaccgccaagacccagagcagagagcagcagttcaacggcacctacagagtggtgagcgtgctgcccatcgagcaccaggactggctgaccggcaaggagttcaagtgcagagtgaaccacatcgacctgcccagccccatcgagagaaccatcagcaaggccagaggcagagcccacaagcccagcgtgtacgtgctgccccccagccccaaggagctgagcagcagcgacaccgtgagcatcacctgcctgatcaaggacttctacccccccgacatcgacgtggagtggcagagcaacggccagcaggagcccgagagaaagcacagaatgacccccccccagctggacgaggacggcagctacttcctgtacagcaagctgagcgtggacaagagcagatggcagcagggcgaccccttcacctgcgccgtgatgcacgagaccctgcagaaccactacaccgacctgagcctgagccacagccccggcaag

SEQ ID NO: 86 - protein, 446 aa, synthetic construct
  REGION 1..446: note = caninized mouse antibody
EVQLVQSGPGLVKPSQSLSLTCVVSGFSLTSYGVHWVRQAPGKGLQWMGWINIYSGIPTYADDFKGRFTFSLDTAKNTAYLQLSSLRAEDTAVYYCARFDGPDYWGQGTLVTVSSASTTAPSVFPLAPSCGSTSGSTVALACLVSGYFPEPVTVSWNSGSLTSGVHTFPSVLQSSGLHSLSSMVTVPSSRWPSETFTCNVVHPASNTKVDKPVFNECRCTDTPPCPVPEPLGGPSVLIFPPKPKDILRITRTPEVTCVVLDLGREDPEVQISWFVDGKEVHTAKTQSREQQFNGTYRVVSVLPIEHQDWLTGKEFKCRVNHIDLPSPIERTISKARGRAHKPSVYVLPPSPKELSSSDTVSITCLIKDFYPPDIDVEWQSNGQQEPERKHRMTPPQLDEDGSYFLYSKLSVDKSRWQQGDPFTCAVMHETLQNHYTDLSLSHSPGK

SEQ ID NO: 87 - DNA, 1338 bp, synthetic construct
  misc_feature 1..1338: note = caninized mouse antibody
  source 1..1338: mol_type = other DNA
gaggtgcagctggtgcagagcggccccggcctggtgaagcccagccagagcctgagcctgacctgcgtggtgagcggcttcagcctgaccagctacggcgtgcactgggtgagacaggcccccggcaagggcctgcagtggatgggctggatcaacatctacagcggcatccccacctacgccgacgacttcaagggcagattcaccttcagcctggacaccgccaagaacaccgcctacctgcagctgagcagcctgagagccgaggacaccgccgtgtactactgcgccagattcgacggccccgactactggggccagggcaccctggtgaccgtgagcagcgccagcaccaccgcccccagcgtgttccccctggcccccagctgcggcagcaccagcggcagcaccgtggccctggcctgcctggtgagcggctacttccccgagcccgtgaccgtgagctggaacagcggcagcctgaccagcggcgtgcacaccttccccagcgtgctgcagagcagcggcctgtacagcctgagcagcaccgtgaccgtgcccagcagcagatggcccagcgagaccttcacctgcaacgtggtgcaccccgccagcaacaccaaggtggacaagcccgtgcccaaggagagcacctgcaagtgcatcagcccctgccccgtgcccgagagcctgggcggccccagcgtgttcatcttcccccccaagcccaaggacatcctgagaatcaccagaacccccgagatcacctgcgtggtgctggacctgggcagagaggaccccgaggtgcagatcagctggttcgtggacggcaaggaggtgcacaccgccaagacccagcccagagagcagcagttcaacagcacctacagagtggtgagcgtgctgcccatcgagcaccaggactggctgaccggcaaggagttcaagtgcagagtgaaccacatcggcctgcccagccccatcgagagaaccatcagcaaggccagaggccaggcccaccagcccagcgtgtacgtgctgccccccagccccaaggagctgagcagcagcgacaccgtgaccctgacctgcctgatcaaggacttcttcccccccgagatcgacgtggagtggcagagcaacggccagcccgagcccgagagcaagtaccacaccaccgccccccagctggacgaggacggcagctacttcctgtacagcaagctgagcgtggacaagagcagatggcagcagggcgacaccttcacctgcgccgtgatgcacgaggccctgcagaaccactacaccgacctgagcctgagccacagccccggcaag

SEQ ID NO: 88 - protein, 446 aa, synthetic construct
  REGION 1..446: note = caninized mouse antibody
EVQLVQSGPGLVKPSQSLSLTCVVSGFSLTSYGVHWVRQAPGKGLQWMGWINIYSGIPTYADDFKGRFTFSLDTAKNTAYLQLSSLRAEDTAVYYCARFDGPDYWGQGTLVTVSSASTTAPSVFPLAPSCGSTSGSTVALACLVSGYFPEPVTVSWNSGSLTSGVHTFPSVLQSSGLYSLSSTVTVPSSRWPSETFTCNVVHPASNTKVDKPVPKESTCKCISPCPVPESLGGPSVFIFPPKPKDILRITRTPEITCVVLDLGREDPEVQISWFVDGKEVHTAKTQPREQQFNSTYRVVSVLPIEHQDWLTGKEFKCRVNHIGLPSPIERTISKARGQAHQPSVYVLPPSPKELSSSDTVTLTCLIKDFFPPEIDVEWQSNGQPEPESKYHTTAPQLDEDGSYFLYSKLSVDKSRWQQGDTFTCAVMHEALQNHYTDLSLSHSPGK

SEQ ID NO: 89 - DNA, 672 bp, synthetic construct
  misc_feature 1..672: note = caninized mouse antibody
  source 1..672: mol_type = other DNA
gacatcgtgatgacccagacccccctgagcctgagcgtgagccccggcgagcccgccagcatgagctgcaagagcagccagagcctgctgaacagcgtgaaccagaagaactacctggcctggtacagacagaagcccggccagagcccccaggtgctggtgtacttcgccagcaccagagtgagcggcgtgcccgacagattcatcggcagcggcagcggcaccgacttcaccctgagaatcagcagagtggaggccgacgacctgggcgtgtactactgccagcagtacttcagcacccccctgaccttcggccagggcaccaagctggagctgaagagaaacgacgcccagcccgccgtgtacctgttccagcccagccccgaccagctgcacaccggcagcgccagcgtggtgtgcctgctgaacagcttctaccccaaggacatcaacgtgaagtggaaggtggacggcgtgatccaggacaccggcatccaggagagcgtgaccgagcaggacagcaaggacagcacctacagcctgagcagcaccctgaccatgagcagcaccgagtacctgagccacgagctgtacagctgcgagatcacccacaagagcctgcccagcaccctgatcaagagcttccagagaagcgagtgccagagagtggac

SEQ ID NO: 90 - protein, 224 aa, synthetic construct
  REGION 1..224: note = caninized mouse antibody
DIVMTQTPLSLSVSPGEPASMSCKSSQSLLNSVNQKNYLAWYRQKPGQSPQVLVYFASTRVSGVPDRFIGSGSGTDFTLRISRVEADDLGVYYCQQYFSTPLTFGQGTKLELKRNDAQPAVYLFQPSPDQLHTGSASVVCLLNSFYPKDINVKWKVDGVIQDTGIQESVTEQDSKDSTYSLSSTLTMSSTEYLSHELYSCEITHKSLPSTLIKSFQRSECQRVD

SEQ ID NO: 91 - DNA, 1338 bp, synthetic construct
  misc_feature 1..1338: note = caninized mouse antibody
  source 1..1338: mol_type = other DNA
gaggtgcagctggtgcagagcggcgccgaggtgaagaagcccggcgccagcgtgaaggtgagctgcaaggccagcggctacaccttcaccacctacggcatgagctgggtgagacaggcccccggcaagggcctgcagtggatgggctggatcaacatctacagcggcatccccacctacgccgacgacttcaagggcagattcgccctgagcctggacaccagcaccagcaccgcctacatggagctgaacagcctgagagccgaggacaccgccgtgtactactgcgccagattcgacggccccgactactggggccagggcaccctggtgaccgtgagcagcgccagcaccaccgcccccagcgtgttccccctggcccccagctgcggcagcaccagcggcagcaccgtggccctggcctgcctggtgagcggctacttccccgagcccgtgaccgtgagctggaacagcggcagcctgaccagcggcgtgcacaccttccccagcgtgctgcagagcagcggcctgcacagcctgagcagcatggtgaccgtgcccagcagcagatggcccagcgagaccttcacctgcaacgtggtgcaccccgccagcaacaccaaggtggacaagcccgtgttcaacgagtgcagatgcaccgacacccccccctgccccgtgcccgagcccctgggcggccccagcgtgctgatcttcccccccaagcccaaggacatcctgagaatcaccagaacccccgaggtgacctgcgtggtgctggacctgggcagagaggaccccgaggtgcagatcagctggttcgtggacggcaaggaggtgcacaccgccaagacccagagcagagagcagcagttcaacggcacctacagagtggtgagcgtgctgcccatcgagcaccaggactggctgaccggcaaggagttcaagtgcagagtgaaccacatcgacctgcccagccccatcgagagaaccatcagcaaggccagaggcagagcccacaagcccagcgtgtacgtgctgccccccagccccaaggagctgagcagcagcgacaccgtgagcatcacctgcctgatcaaggacttctacccccccgacatcgacgtggagtggcagagcaacggccagcaggagcccgagagaaagcacagaatgacccccccccagctggacgaggacggcagctacttcctgtacagcaagctgagcgtggacaagagcagatggcagcagggcgaccccttcacctgcgccgtgatgcacgagaccctgcagaaccactacaccgacctgagcctgagccacagccccggcaag

SEQ ID NO: 92 - protein, 446 aa, synthetic construct
  REGION 1..446: note = caninized mouse antibody
EVQLVQSGAEVKKPGASVKVSCKASGYTFTTYGMSWVRQAPGKGLQWMGWINIYSGIPTYADDFKGRFALSLDTSTSTAYMELNSLRAEDTAVYYCARFDGPDYWGQGTLVTVSSASTTAPSVFPLAPSCGSTSGSTVALACLVSGYFPEPVTVSWNSGSLTSGVHTFPSVLQSSGLHSLSSMVTVPSSRWPSETFTCNVVHPASNTKVDKPVFNECRCTDTPPCPVPEPLGGPSVLIFPPKPKDILRITRTPEVTCVVLDLGREDPEVQISWFVDGKEVHTAKTQSREQQFNGTYRVVSVLPIEHQDWLTGKEFKCRVNHIDLPSPIERTISKARGRAHKPSVYVLPPSPKELSSSDTVSITCLIKDFYPPDIDVEWQSNGQQEPERKHRMTPPQLDEDGSYFLYSKLSVDKSRWQQGDPFTCAVMHETLQNHYTDLSLSHSPGK

SEQ ID NO: 93 - DNA, 1338 bp, synthetic construct
  misc_feature 1..1338: note = caninized mouse antibody
  source 1..1338: mol_type = other DNA
gaggtgcagctggtgcagagcggcgccgaggtgaagaagcccggcgccagcgtgaaggtgagctgcaaggccagcggctacaccttcaccacctacggcatgagctgggtgagacaggcccccggcaagggcctgcagtggatgggctggatcaacatctacagcggcatccccacctacgccgacgacttcaagggcagattcgccctgagcctggacaccagcaccagcaccgcctacatggagctgaacagcctgagagccgaggacaccgccgtgtactactgcgccagattcgacggccccgactactggggccagggcaccctggtgaccgtgagcagcgccagcaccaccgcccccagcgtgttccccctggcccccagctgcggcagcaccagcggcagcaccgtggccctggcctgcctggtgagcggctacttccccgagcccgtgaccgtgagctggaacagcggcagcctgaccagcggcgtgcacaccttccccagcgtgctgcagagcagcggcctgtacagcctgagcagcaccgtgaccgtgcccagcagcagatggcccagcgagaccttcacctgcaacgtggtgcaccccgccagcaacaccaaggtggacaagcccgtgcccaaggagagcacctgcaagtgcatcagcccctgccccgtgcccgagagcctgggcggccccagcgtgttcatcttcccccccaagcccaaggacatcctgagaatcaccagaacccccgagatcacctgcgtggtgctggacctgggcagagaggaccccgaggtgcagatcagctggttcgtggacggcaaggaggtgcacaccgccaagacccagcccagagagcagcagttcaacagcacctacagagtggtgagcgtgctgcccatcgagcaccaggactggctgaccggcaaggagttcaagtgcagagtgaaccacatcggcctgcccagccccatcgagagaaccatcagcaaggccagaggccaggcccaccagcccagcgtgtacgtgctgccccccagccccaaggagctgagcagcagcgacaccgtgaccctgacctgcctgatcaaggacttcttcccccccgagatcgacgtggagtggcagagcaacggccagcccgagcccgagagcaagtaccacaccaccgccccccagctggacgaggacggcagctacttcctgtacagcaagctgagcgtggacaagagcagatggcagcagggcgacaccttcacctgcgccgtgatgcacgaggccctgcagaaccactacaccgacctgagcctgagccacagccccggcaag

SEQ ID NO: 94 - protein, 446 aa, synthetic construct
  REGION 1..446: note = caninized mouse antibody
EVQLVQSGAEVKKPGASVKVSCKASGYTFTTYGMSWVRQAPGKGLQWMGWINIYSGIPTYADDFKGRFALSLDTSTSTAYMELNSLRAEDTAVYYCARFDGPDYWGQGTLVTVSSASTTAPSVFPLAPSCGSTSGSTVALACLVSGYFPEPVTVSWNSGSLTSGVHTFPSVLQSSGLYSLSSTVTVPSSRWPSETFTCNVVHPASNTKVDKPVPKESTCKCISPCPVPESLGGPSVFIFPPKPKDILRITRTPEITCVVLDLGREDPEVQISWFVDGKEVHTAKTQPREQQFNSTYRVVSVLPIEHQDWLTGKEFKCRVNHIGLPSPIERTISKARGQAHQPSVYVLPPSPKELSSSDTVTLTCLIKDFFPPEIDVEWQSNGQPEPESKYHTTAPQLDEDGSYFLYSKLSVDKSRWQQGDTFTCAVMHEALQNHYTDLSLSHSPGK

SEQ ID NO: 95 - DNA, 672 bp, synthetic construct; identical to SEQ ID NO: 89
  misc_feature 1..672: note = caninized mouse antibody
  source 1..672: mol_type = other DNA

SEQ ID NO: 96 - protein, 224 aa, synthetic construct; identical to SEQ ID NO: 90
  REGION 1..224: note = caninized mouse antibody

SEQ ID NO: 97 - DNA, 1353 bp, synthetic construct
  misc_feature 1..1353: note = caninized mouse antibody
  source 1..1353: mol_type = other DNA
gaggtgcagctggtgcagagcgtggccgagctggtgaagcccggcgccagcgtgaaggtgagctgcaccgtgagcggcttcaacatcaagaacacctacatgcactgggtgagacaggcccccggcaagggcctgcagtggatcggcagaatcgaccccgccaacgtgaacaccaagtacgcccccaagttccagggcagagccaccatcaccgccgacaccagcaccaacaccgcctacatgcagctgagcagcctgagagccgaggacaccgccgtgtactactgcgccagaatcttctacgactacgacggcgacatcgacgtgtggggccagggcaccctggtgaccgtgagcagcgccagcaccaccgcccccagcgtgttccccctggcccccagctgcggcagcaccagcggcagcaccgtggccctggcctgcctggtgagcggctacttccccgagcccgtgaccgtgagctggaacagcggcagcctgaccagcggcgtgcacaccttccccagcgtgctgcagagcagcggcctgcacagcctgagcagcatggtgaccgtgcccagcagcagatggcccagcgagaccttcacctgcaacgtggtgcaccccgccagcaacaccaaggtggacaagcccgtgttcaacgagtgcagatgcaccgacacccccccctgccccgtgcccgagcccctgggcggccccagcgtgctgatcttcccccccaagcccaaggacatcctgagaatcaccagaacccccgaggtgacctgcgtggtgctggacctgggcagagaggaccccgaggtgcagatcagctggttcgtggacggcaaggaggtgcacaccgccaagacccagagcagagagcagcagttcaacggcacctacagagtggtgagcgtgctgcccatcgagcaccaggactggctgaccggcaaggagttcaagtgcagagtgaaccacatcgacctgcccagccccatcgagagaaccatcagcaaggccagaggcagagcccacaagcccagcgtgtacgtgctgccccccagccccaaggagctgagcagcagcgacaccgtgagcatcacctgcctgatcaaggacttctacccccccgacatcgacgtggagtggcagagcaacggccagcaggagcccgagagaaagcacagaatgacccccccccagctggacgaggacggcagctacttcctgtacagcaagctgagcgtggacaagagcagatggcagcagggcgaccccttcacctgcgccgtgatgcacgagaccctgcagaaccactacaccgacctgagcctgagccacagccccggcaag

SEQ ID NO: 98 - protein, 451 aa, synthetic construct
  REGION 1..451: note = caninized mouse antibody
EVQLVQSVAELVKPGASVKVSCTVSGFNIKNTYMHWVRQAPGKGLQWIGRIDPANVNTKYAPKFQGRATITADTSTNTAYMQLSSLRAEDTAVYYCARIFYDYDGDIDVWGQGTLVTVSSASTTAPSVFPLAPSCGSTSGSTVALACLVSGYFPEPVTVSWNSGSLTSGVHTFPSVLQSSGLHSLSSMVTVPSSRWPSETFTCNVVHPASNTKVDKPVFNECRCTDTPPCPVPEPLGGPSVLIFPPKPKDILRITRTPEVTCVVLDLGREDPEVQISWFVDGKEVHTAKTQSREQQFNGTYRVVSVLPIEHQDWLTGKEFKCRVNHIDLPSPIERTISKARGRAHKPSVYVLPPSPKELSSSDTVSITCLIKDFYPPDIDVEWQSNGQQEPERKHRMTPPQLDEDGSYFLYSKLSVDKSRWQQGDPFTCAVMHETLQNHYTDLSLSHSPGK

SEQ ID NO: 99 - DNA, 1353 bp, synthetic construct
  misc_feature 1..1353: note = caninized mouse antibody
  source 1..1353: mol_type = other DNA
gaggtgcagctggtgcagagcgtggccgagctggtgaagcccggcgccagcgtgaaggtgagctgcaccgtgagcggcttcaacatcaagaacacctacatgcactgggtgagacaggcccccggcaagggcctgcagtggatcggcagaatcgaccccgccaacgtgaacaccaagtacgcccccaagttccagggcagagccaccatcaccgccgacaccagcaccaacaccgcctacatgcagctgagcagcctgagagccgaggacaccgccgtgtactactgcgccagaatcttctacgactacgacggcgacatcgacgtgtggggccagggcaccctggtgaccgtgagcagcgccagcaccaccgcccccagcgtgttccccctggcccccagctgcggcagcaccagcggcagcaccgtggccctggcctgcctggtgagcggctacttccccgagcccgtgaccgtgagctggaacagcggcagcctgaccagcggcgtgcacaccttccccagcgtgctgcagagcagcggcctgtacagcctgagcagcaccgtgaccgtgcccagcagcagatggcccagcgagaccttcacctgcaacgtggtgcaccccgccagcaacaccaaggtggacaagcccgtgcccaaggagagcacctgcaagtgcatcagcccctgccccgtgcccgagagcctgggcggccccagcgtgttcatcttcccccccaagcccaaggacatcctgagaatcaccagaacccccgagatcacctgcgtggtgctggacctgggcagagaggaccccgaggtgcagatcagctggttcgtggacggcaaggaggtgcacaccgccaagacccagcccagagagcagcagttcaacagcacctacagagtggtgagcgtgctgcccatcgagcaccaggactggctgaccggcaaggagttcaagtgcagagtgaaccacatcggcctgcccagccccatcgagagaaccatcagcaaggccagaggccaggcccaccagcccagcgtgtacgtgctgccccccagccccaaggagctgagcagcagcgacaccgtgaccctgacctgcctgatcaaggacttcttcccccccgagatcgacgtggagtggcagagcaacggccagcccgagcccgagagcaagtaccacaccaccgccccccagctggacgaggacggcagctacttcctgtacagcaagctgagcgtggacaagagcagatggcagcagggcgacaccttcacctgcgccgtgatgcacgaggccctgcagaaccactacaccgacctgagcctgagccacagccccggcaag

SEQ ID NO: 100 - protein, 451 aa, synthetic construct
  REGION 1..451: note = caninized mouse antibody
EVQLVQSVAELVKPGASVKVSCTVSGFNIKNTYMHWVRQAPGKGLQWIGRIDPANVNTKYAPKFQGRATITADTSTNTAYMQLSSLRAEDTAVYYCARIFYDYDGDIDVWGQGTLVTVSSASTTAPSVFPLAPSCGSTSGSTVALACLVSGYFPEPVTVSWNSGSLTSGVHTFPSVLQSSGLYSLSSTVTVPSSRWPSETFTCNVVHPASNTKVDKPVPKESTCKCISPCPVPESLGGPSVFIFPPKPKDILRITRTPEITCVVLDLGREDPEVQISWFVDGKEVHTAKTQPREQQFNSTYRVVSVLPIEHQDWLTGKEFKCRVNHIGLPSPIERTISKARGQAHQPSVYVLPPSPKELSSSDTVTLTCLIKDFFPPEIDVEWQSNGQPEPESKYHTTAPQLDEDGSYFLYSKLSVDKSRWQQGDTFTCAVMHEALQNHYTDLSLSHSPGK

SEQ ID NO: 101 - DNA, 654 bp, synthetic construct
  misc_feature 1..654: note = caninized mouse antibody
  source 1..654: mol_type = other DNA
gacatcgtgatgacccagacccccctgagcctgagcgtgagcctgggcgagcccgccagcatcagctgccacgccagccagaacatcaacgtgtggctgagctggtacagacagaagcccggccagatcccccagctgctgatctacaaggccagcaacctgcacaccggcgtgcccgacagattcagcggcagcggcagcggcaccgacttcaccctgagaatcagcagagtggaggccgacgacgccggcgtgtactactgccagcagggccagagctaccccctgaccttcggccagggcaccaaggtggagatcaagagaaacgacgcccagcccgccgtgtacctgttccagcccagccccgaccagctgcacaccggcagcgccagcgtggtgtgcctgctgaacagcttctaccccaaggacatcaacgtgaagtggaaggtggacggcgtgatccaggacaccggcatccaggagagcgtgaccgagcaggacagcaaggacagcacctacagcctgagcagcaccctgaccatgagcagcaccgagtacctgagccacgagctgtacagctgcgagatcacccacaagagcctgcccagcaccctgatcaagagcttccagagaagcgagtgccagagagtggac

SEQ ID NO: 102 - protein, 218 aa, synthetic construct
  REGION 1..218: note = caninized mouse antibody
DIVMTQTPLSLSVSLGEPASISCHASQNINVWLSWYRQKPGQIPQLLIYKASNLHTGVPDRFSGSGSGTDFTLRISRVEADDAGVYYCQQGQSYPLTFGQGTKVEIKRNDAQPAVYLFQPSPDQLHTGSASVVCLLNSFYPKDINVKWKVDGVIQDTGIQESVTEQDSKDSTYSLSSTLTMSSTEYLSHELYSCEITHKSLPSTLIKSFQRSECQRVD

SEQ ID NO: 103 - DNA, 1338 bp, synthetic construct
  misc_feature 1..1338: note = caninized mouse antibody
  source 1..1338: mol_type = other DNA
gaggtgcagctggtgcagagcggcgccgaggtgaagaagcccggcgccagcgtgaaggtgagctgcaaggccagcggctacaccttcaccacctacggcatgagctgggtgagacaggcccccggcaagggcctgcagtggatgggctggatcaacatctacagcggcatgcccacctacgccgacgacttcaagggcagattcgccctgagcctggacaccagcaccagcaccgcctacatggagctgaacagcctgagagccgaggacaccgccgtgtactactgcaccagattcgacggccccgactactggggccagggcaccctggtgaccgtgagcagcgccagcaccaccgcccccagcgtgttccccctggcccccagctgcggcagcaccagcggcagcaccgtggccctggcctgcctggtgagcggctacttccccgagcccgtgaccgtgagctggaacagcggcagcctgaccagcggcgtgcacaccttccccagcgtgctgcagagcagcggcctgcacagcctgagcagcatggtgaccgtgcccagcagcagatggcccagcgagaccttcacctgcaacgtggtgcaccccgccagcaacaccaaggtggacaagcccgtgttcaacgagtgcagatgcaccgacacccccccctgccccgtgcccgagcccctgggcggccccagcgtgctgatcttcccccccaagcccaaggacatcctgagaatcaccagaacccccgaggtgacctgcgtggtgctggacctgggcagagaggaccccgaggtgcagatcagctggttcgtggacggcaaggaggtgcacaccgccaagacccagagcagagagcagcagttcaacggcacctacagagtggtgagcgtgctgcccatcgagcaccaggactggctgaccggcaaggagttcaagtgcagagtgaaccacatcgacctgcccagccccatcgagagaaccatcagcaaggccagaggcagagcccacaagcccagcgtgtacgtgctgccccccagccccaaggagctgagcagcagcgacaccgtgagcatcacctgcctgatcaaggacttctacccccccgacatcgacgtggagtggcagagcaacggccagcaggagcccgagagaaagcacagaatgacccccccccagctggacgaggacggcagctacttcctgtacagcaagctgagcgtggacaagagcagatggcagcagggcgaccccttcacctgcgccgtgatgcacgagaccctgcagaaccactacaccgacctgagcctgagccacagccccggcaag

SEQ ID NO: 104 - protein, 446 aa, synthetic construct
  REGION 1..446: note = caninized mouse antibody
EVQLVQSGAEVKKPGASVKVSCKASGYTFTTYGMSWVRQAPGKGLQWMGWINIYSGMPTYADDFKGRFALSLDTSTSTAYMELNSLRAEDTAVYYCTRFDGPDYWGQGTLVTVSSASTTAPSVFPLAPSCGSTSGSTVALACLVSGYFPEPVTVSWNSGSLTSGVHTFPSVLQSSGLHSLSSMVTVPSSRWPSETFTCNVVHPASNTKVDKPVFNECRCTDTPPCPVPEPLGGPSVLIFPPKPKDILRITRTPEVTCVVLDLGREDPEVQISWFVDGKEVHTAKTQSREQQFNGTYRVVSVLPIEHQDWLTGKEFKCRVNHIDLPSPIERTISKARGRAHKPSVYVLPPSPKELSSSDTVSITCLIKDFYPPDIDVEWQSNGQQEPERKHRMTPPQLDEDGSYFLYSKLSVDKSRWQQGDPFTCAVMHETLQNHYTDLSLSHSPGK

SEQ ID NO: 105 - DNA, 1338 bp, synthetic construct
  misc_feature 1..1338: note = caninized mouse antibody
  source 1..1338: mol_type = other DNA
gaggtgcagctggtgcagagcggcgccgaggtgaagaagcccggcgccagcgtgaaggtgagctgcaaggccagcggctacaccttcaccacctacggcatgagctgggtgagacaggcccccggcaagggcctgcagtggatgggctggatcaacatctacagcggcatgcccacctacgccgacgacttcaagggcagattcgccctgagcctggacaccagcaccagcaccgcctacatggagctgaacagcctgagagccgaggacaccgccgtgtactactgcaccagattcgacggccccgactactggggccagggcaccctggtgaccgtgagcagcgccagcaccaccgcccccagcgtgttccccctggcccccagctgcggcagcaccagcggcagcaccgtggccctggcctgcctggtgagcggctacttccccgagcccgtgaccgtgagctggaacagcggcagcctgaccagcggcgtgcacaccttccccagcgtgctgcagagcagcggcctgtacagcctgagcagcaccgtgaccgtgcccagcagcagatggcccagcgagaccttcacctgcaacgtggtgcaccccgccagcaacaccaaggtggacaagcccgtgcccaaggagagcacctgcaagtgcatcagcccctgccccgtgcccgagagcctgggcggccccagcgtgttcatcttcccccccaagcccaaggacatcctgagaatcaccagaacccccgagatcacctgcgtggtgctggacctgggcagagaggaccccgaggtgcagatcagctggttcgtggacggcaaggaggtgcacaccgccaagacccagcccagagagcagcagttcaacagcacctacagagtggtgagcgtgctgcccatcgagcaccaggactggctgaccggcaaggagttcaagtgcagagtgaaccacatcggcctgcccagccccatcgagagaaccatcagcaaggccagaggccaggcccaccagcccagcgtgtacgtgctgccccccagccccaaggagctgagcagcagcgacaccgtgaccctgacctgcctgatcaaggacttcttcccccccgagatcgacgtggagtggcagagcaacggccagcccgagcccgagagcaagtaccacaccaccgccccccagctggacgaggacggcagctacttcctgtacagcaagctgagcgtggacaagagcagatggcagcagggcgacaccttcacctgcgccgtgatgcacgaggccctgcagaaccactacaccgacctgagcctgagccacagccccggcaag

SEQ ID NO: 106 - protein, 446 aa, synthetic construct
  REGION 1..446: note = caninized mouse antibody
EVQLVQSGAEVKKPGASVKVSCKASGYTFTTYGMSWVRQAPGKGLQWMGWINIYSGMPTYADDFKGRFALSLDTSTSTAYMELNSLRAEDTAVYYCTRFDGPDYWGQGTLVTVSSASTTAPSVFPLAPSCGSTSGSTVALACLVSGYFPEPVTVSWNSGSLTSGVHTFPSVLQSSGLYSLSSTVTVPSSRWPSETFTCNVVHPASNTKVDKPVPKESTCKCISPCPVPESLGGPSVFIFPPKPKDILRITRTPEITCVVLDLGREDPEVQISWFVDGKEVHTAKTQPREQQFNSTYRVVSVLPIEHQDWLTGKEFKCRVNHIGLPSPIERTISKARGQAHQPSVYVLPPSPKELSSSDTVTLTCLIKDFFPPEIDVEWQSNGQPEPESKYHTTAPQLDEDGSYFLYSKLSVDKSRWQQGDTFTCAVMHEALQNHYTDLSLSHSPGK

SEQ ID NO: 107 - DNA, 672 bp, synthetic construct
  misc_feature 1..672: note = caninized mouse antibody
  source 1..672: mol_type = other DNA
gacatcgtgatgacccagacccccctgagcctgagcgtgagccccggcgagcccgccagcatgagctgcaagagcagccagagcctgctgaacagcgtgaaccagaagaactacctggcctggtacagacagaagcccggccagagcccccaggtgctggtgtacttcgccagcaccagaatcagcggcgtgcccgacagattcatcggcagcggcagcggcaccgacttcaccctgagaatcagcagagtggaggccgacgacctgggcgtgtactactgccagcagtacttcagcacccccctgaccttcggccagggcaccaagctggagctgaagagaaacgacgcccagcccgccgtgtacctgttccagcccagccccgaccagctgcacaccggcagcgccagcgtggtgtgcctgctgaacagcttctaccccaaggacatcaacgtgaagtggaaggtggacggcgtgatccaggacaccggcatccaggagagcgtgaccgagcaggacagcaaggacagcacctacagcctgagcagcaccctgaccatgagcagcaccgagtacctgagccacgagctgtacagctgcgagatcacccacaagagcctgcccagcaccctgatcaagagcttccagagaagcgagtgccagagagtggac

SEQ ID NO: 108 - protein, 224 aa, synthetic construct
  REGION 1..224: note = caninized mouse antibody
DIVMTQTPLSLSVSPGEPASMSCKSSQSLLNSVNQKNYLAWYRQKPGQSPQVLVYFASTRISGVPDRFIGSGSGTDFTLRISRVEADDLGVYYCQQYFSTPLTFGQGTKLELKRNDAQPAVYLFQPSPDQLHTGSASVVCLLNSFYPKDINVKWKVDGVIQDTGIQESVTEQDSKDSTYSLSSTLTMSSTEYLSHELYSCEITHKSLPSTLIKSFQRSECQRVD

SEQ ID NO: 109 - protein, 17 aa, Canis lupus
  source 1..17: note = Canis familiaris
FNECRCTDTPPCPVPEP

SEQ ID NO: 110 - protein, 22 aa, Canis lupus
  source 1..22: note = Canis familiaris
PKRENGRVPRPPDCPKCPAPEM

SEQ ID NO: 111 - protein, 20 aa, Canis lupus
  source 1..20: note = Canis familiaris
AKECECKCNCNNCPCPGCGL

SEQ ID NO: 112 - protein, 17 aa, synthetic construct
  REGION 1..17: note = modified canine
PKESTCKCIPPCPVPES

SEQ ID NO: 113 - DNA, 795 bp, Canis lupus
  source 1..795: mol_type = unassigned DNA; note = Canis familiaris
ctagactcccctgacaggccctggagcccgctcaccttctccccggcgcagctcacggtgcaggagggagagaacgccacgttcacctgcagcctggccgacatccccgacagcttcgtgctcaactggtaccgcctgagcccccgcaaccagacggacaagctggccgccttccaggaggaccgcatcgagccgggccgggacaggcgcttccgcgtcatgcggctgcccaacgggcgggacttccacatgagcatcgtcgctgcgcgcctcaacgacagcggcatctacctgtgcggggccatctacctgccccccaacacacagatcaacgagagtccccgcgcagagctctccgtgacggagagaaccctggagccccccacacagagccccagccccccacccagactcagcggccagttgcaggggctggtcatcggcgtcacgagcgtgctggtgggtgtcctgctactgctgctgctgacctgggtcctggccgctgtcttccccagggccacccgaggtgcctgtgtgtgcgggagcgaggacgagcctctgaaggagggccccgatgcagcgcccgtcttcaccctggactacggggagctggacttccagtggcgagagaagacgccggagcccccggcgccctgtgccccggagcagaccgagtatgccaccatcgtcttcccgggcaggccggcgtccccgggccgcagggcctcggccagcagcctgcagggagcccagcctccgagccccgaggacggacccggcctgtggcccctctga

SEQ ID NO: 114 - protein, 264 aa, Canis lupus
  source 1..264: note = Canis familiaris
LDSPDRPWSPLTFSPAQLTVQEGENATFTCSLADIPDSFVLNWYRLSPRNQTDKLAAFQEDRIEPGRDRRFRVMRLPNGRDFHMSIVAARLNDSGIYLCGAIYLPPNTQINESPRAELSVTERTLEPPTQSPSPPPRLSGQLQGLVIGVTSVLVGVLLLLLLTWVLAAVFPRATRGACVCGSEDEPLKEGPDAAPVFTLDYGELDFQWREKTPEPPAPCAPEQTEYATIVFPGRPASPGRRASASSLQGAQPPSPEDGPGLWPL

SEQ ID NO: 115 - DNA, 438 bp, Canis lupus
  source 1..438: mol_type = unassigned DNA; note = Canis familiaris
ctggattcccccgacagaccctggagccctctcaccttctcccctgcccagctgaccgtccaggaaggcgagaatgccaccttcacctgcagcctcgccgacatccccgacagcttcgtgctgaactggtacagactgagccccaggaaccagaccgacaagctggccgctttccaggaggacaggatcgaacccggcagggacaggaggtttagggtcatgaggctgcccaacggcagggacttccacatgtccatcgtggccgccagactgaacgactccggcatctacctgtgcggcgctatctacctgccccccaacacccagatcaacgagagccccagggccgaactgagcgtgacagagagaaccctggaacctcccacccagagcccttcccctcctcctagactgagcggacagctgcagggcctggtg

SEQ ID NO: 116 - protein, 146 aa, Canis lupus
  source 1..146: note = Canis familiaris
LDSPDRPWSPLTFSPAQLTVQEGENATFTCSLADIPDSFVLNWYRLSPRNQTDKLAAFQEDRIEPGRDRRFRVMRLPNGRDFHMSIVAARLNDSGIYLCGAIYLPPNTQINESPRAELSVTERTLEPPTQSPSPPPRLSGQLQGLV

SEQ ID NO: 117 - DNA, 1128 bp, synthetic construct
  misc_feature 1..1128: note = canine and human sequence
  source 1..1128: mol_type = other DNA
ctggattcccccgacagaccctggagccctctcaccttctcccctgcccagctgaccgtccaggaaggcgagaatgccaccttcacctgcagcctcgccgacatccccgacagcttcgtgctgaactggtacagactgagccccaggaaccagaccgacaagctggccgctttccaggaggacaggatcgaacccggcagggacaggaggtttagggtcatgaggctgcccaacggcagggacttccacatgtccatcgtggccgccagactgaacgactccggcatctacctgtgcggcgctatctacctgccccccaacacccagatcaacgagagccccagggccgaactgagcgtgacagagagaaccctggaacctcccacccagagcccttcccctcctcctagactgagcggacagctgcagggcctggtgggtaccgacaaaactcacacatgcccaccgtgcccagcacctgaactcctggggggaccgtcagtcttcctcttccccccaaaacccaaggacaccctcatgatctcccggacccctgaggtcacatgcgtggtggtggacgtgagccacgaagaccctgaggtcaagttcaactggtacgtggacggcgtggaggtgcataatgccaagacaaagccgcgggaggagcagtacaacagcacgtaccgtgtggtcagcgtcctcaccgtcctgcaccaggactggctgaatggcaaggagtacaagtgcaaggtctccaacaaagccctcccagcccccatcgagaaaaccatctccaaagccaaagggcagccccgagaaccacaggtgtacaccctgcccccatcccgggatgagctgaccaagaaccaggtcagcctgacctgcctggtcaaaggcttctatcccagcgacatcgccgtggagtgggagagcaatgggcagccggagaacaactacaagaccacgcctcccgtgctggactccgacggctccttcttcctctacagcaagctcaccgtggacaagagcaggtggcagcaggggaacgtcttctcatgctccgtgatgcatgaggctctgcacaaccactacacgcagaagagcctctccctgtctccgggtaaatga

SEQ ID NO: 118 - protein, 375 aa, synthetic construct
  REGION 1..375: note = canine and human sequence
LDSPDRPWSPLTFSPAQLTVQEGENATFTCSLADIPDSFVLNWYRLSPRNQTDKLAAFQEDRIEPGRDRRFRVMRLPNGRDFHMSIVAARLNDSGIYLCGAIYLPPNTQINESPRAELSVTERTLEPPTQSPSPPPRLSGQLQGLVGTDKTHTCPPCPAPELLGGPSVFLFPPKPKDTLMISRTPEVTCVVVDVSHEDPEVKFNWYVDGVEVHNAKTKPREEQYNSTYRVVSVLTVLHQDWLNGKEYKCKVSNKALPAPIEKTISKAKGQPREPQVYTLPPSRDELTKNQVSLTCLVKGFYPSDIAVEWESNGQPENNYKTTPPVLDSDGSFFLYSKLTVDKSRWQQGNVFSCSVMHEALHNHYTQKSLSLSPGK

SEQ ID NO: 119 - DNA, 816 bp, Canis lupus
  source 1..816: mol_type = unassigned DNA; note = Canis familiaris
tttacgatcacagtttctaaggacctgtatgtggtagagtatggtggcaatgtgacaatggaatgcaaattcccggtggaaaaacagttaaacttgtttgcactaatcgtctactgggaaatggaggataaaaaaattatacaatttgtgaatggaaaggaagacctgaaagttcagcacagcagctacagccagagggctcagctattgaaggaccagctcttcttggggaaggctgcgcttcagatcacagatgtgagattgcaggatgcaggggtttactgctgcttgatcggctatggcggtgctgactacaagcggattactttgaaagttcatgccccgtaccgcaacatcagccaaagaatttctgtggatcctgtcacctctgaacatgaactaatgtgtcaggctgagggttaccctgaggctgaagtcatctggacaagcagtgaccaccgagtcctgagtggcaaaaccaccatcactaattccaatagggaagagaagcttttcaatgtgaccagcacgctgaacatcaatgcaacagctaatgagattttctactgcacttttcaaagatcaggtcctgaggaaaacaatactgccgagttggtcatcccagaacgactgcccgttccagcaagtgagaggactcatttcatgattctgggacctttcctgttgcttcttggtgtagtcctggcagtcactttctgtctaaaaaaacatgggagaatgatggatgtggaaaaatgttgcacccgagataggaactcaaagaaacgaaatgatatacaatttgaagagacataa

SEQ ID NO: 120 - protein, 271 aa, Canis lupus
  source 1..271: note = Canis familiaris
FTITVSKDLYVVEYGGNVTMECKFPVEKQLNLFALIVYWEMEDKKIIQFVNGKEDLKVQHSSYSQRAQLLKDQLFLGKAALQITDVRLQDAGVYCCLIGYGGADYKRITLKVHAPYRNISQRISVDPVTSEHELMCQAEGYPEAEVIWTSSDHRVLSGKTTITNSNREEKLFNVTSTLNINATANEIFYCTFQRSGPEENNTAELVIPERLPVPASERTHFMILGPFLLLLGVVLAVTFCLKKHGRMMDVEKCCTRDRNSKKRNDIQFEET

SEQ ID NO: 121 - DNA, 660 bp, Canis lupus
  source 1..660: mol_type = unassigned DNA; note = Canis familiaris
tttaccatcaccgtgtccaaggacctgtacgtggtcgagtacggcggcaatgtgaccatggagtgcaagttccccgtggagaagcagctgaacctgttcgccctcatcgtgtactgggagatggaggacaagaagatcatccagttcgtgaacggcaaggaggacctgaaggtgcagcactccagctactcccagagagcccagctgctgaaggaccagctgttcctgggcaaggccgccctgcagatcaccgacgtgagactgcaggacgccggcgtgtattgctgcctgatcggctacggaggcgccgactacaagaggatcaccctgaaggtgcatgcaccctacaggaacatcagccagaggatcagcgtcgatcccgtgaccagcgagcacgagctgatgtgccaagccgagggctatcccgaggccgaagtgatctggaccagcagcgaccacagggtcctgagcggcaagaccaccatcaccaacagcaacagggaggagaagctgttcaacgtgaccagcaccctcaacatcaacgccaccgccaacgagatcttctactgcaccttccagaggagcggccccgaagagaacaacaccgccgagctggtgatccccgagagactgcctgtgcctgccagcgagaggacccac

SEQ ID NO: 122 - protein, 220 aa, Canis lupus
  source 1..220: note = Canis familiaris
FTITVSKDLYVVEYGGNVTMECKFPVEKQLNLFALIVYWEMEDKKIIQFVNGKEDLKVQHSSYSQRAQLLKDQLFLGKAALQITDVRLQDAGVYCCLIGYGGADYKRITLKVHAPYRNISQRISVDPVTSEHELMCQAEGYPEAEVIWTSSDHRVLSGKTTITNSNREEKLFNVTSTLNINATANEIFYCTFQRSGPEENNTAELVIPERLPVPASERTH

SEQ ID NO: 123 - DNA, 1350 bp, Canis lupus
  source 1..1350: mol_type = unassigned DNA; note = Canis familiaris
tttaccatcaccgtgtccaaggacctgtacgtggtcgagtacggcggcaatgtgaccatggagtgcaagttccccgtggagaagcagctgaacctgttcgccctcatcgtgtactgggagatggaggacaagaagatcatccagttcgtgaacggcaaggaggacctgaaggtgcagcactccagctactcccagagagcccagctgctgaaggaccagctgttcctgggcaaggccgccctgcagatcaccgacgtgagactgcaggacgccggcgtgtattgctgcctgatcggctacggaggcgccgactacaagaggatcaccctgaaggtgcatgcaccctacaggaacatcagccagaggatcagcgtcgatcccgtgaccagcgagcacgagctgatgtgccaagccgagggctatcccgaggccgaagtgatctggaccagcagcgaccacagggtcctgagcggcaagaccaccatcaccaacagcaacagggaggagaagctgttcaacgtgaccagcaccctcaacatcaacgccaccgccaacgagatcttctactgcaccttccagaggagcggccccgaagagaacaacaccgccgagctggtgatccccgagagactgcctgtgcctgccagcgagaggacccacggtaccgacaaaactcacacatgcccaccgtgcccagcacctgaactcctggggggaccgtcagtcttcctcttccccccaaaacccaaggacaccctcatgatctcccggacccctgaggtcacatgcgtggtggtggacgtgagccacgaagaccctgaggtcaagttcaactggtacgtggacggcgtggaggtgcataatgccaagacaaagccgcgggaggagcagtacaacagcacgtaccgtgtggtcagcgtcctcaccgtcctgcaccaggactggctgaatggcaaggagtacaagtgcaaggtctccaacaaagccctcccagcccccatcgagaaaaccatctccaaagccaaagggcagccccgagaaccacaggtgtacaccctgcccccatcccgggatgagctgaccaagaaccaggtcagcctgacctgcctggtcaaaggcttctatcccagcgacatcgccgtggagtgggagagcaatgggcagccggagaacaactacaagaccacgcctcccgtgctggactccgacggctccttcttcctctacagcaagctcaccgtggacaagagcaggtggcagcaggggaacgtcttctcatgctccgtgatgcatgaggctctgcacaaccactacacgcagaagagcctctccctgtctccgggtaaatga

SEQ ID NO: 124 - protein, 449 aa, Canis lupus
  source 1..449: note = Canis familiaris
FTITVSKDLYVVEYGGNVTMECKFPVEKQLNLFALIVYWEMEDKKIIQFVNGKEDLKVQHSSYSQRAQLLKDQLFLGKAALQITDVRLQDAGVYCCLIGYGGADYKRITLKVHAPYRNISQRISVDPVTSEHELMCQAEGYPEAEVIWTSSDHRVLSGKTTITNSNREEKLFNVTSTLNINATANEIFYCTFQRSGPEENNTAELVIPERLPVPASERTHGTDKTHTCPPCPAPELLGGPSVFLFPPKPKDTLMISRTPEVTCVVVDVSHEDPEVKFNWYVDGVEVHNAKTKPREEQYNSTYRVVSVLTVLHQDWLNGKEYKCKVSNKALPAPIEKTISKAKGQPREPQVYTLPPSRDELTKNQVSLTCLVKGFYPSDIAVEWESNGQPENNYKTTPPVLDSDGSFFLYSKLTVDKSRWQQGNVFSCSVMHEALHNHYTQKSLSLSPGK

SEQ ID NO: 125 - DNA, 648 bp, Canis lupus
  source 1..648: mol_type = unassigned DNA; note = Canis familiaris
ctgggcggccccagcgtgctgatcttcccccccaagcccaaggacatcctgagaatcaccagaacccccgaggtgacctgcgtggtgctggacctgggcagagaggaccccgaggtgcagatcagctggttcgtggacggcaaggaggtgcacaccgccaagacccagagcagagagcagcagttcaacggcacctacagagtggtgagcgtgctgcccatcgagcaccaggactggctgaccggcaaggagttcaagtgcagagtgaaccacatcgacctgcccagccccatcgagagaaccatcagcaaggccagaggcagagcccacaagcccagcgtgtacgtgctgccccccagccccaaggagctgagcagcagcgacaccgtgagcatcacctgcctgatcaaggacttctacccccccgacatcgacgtggagtggcagagcaacggccagcaggagcccgagagaaagcacagaatgacccccccccagctggacgaggacggcagctacttcctgtacagcaagctgagcgtggacaagagcagatggcagcagggcgaccccttcacctgcgccgtgatgcacgagaccctgcagaaccactacaccgacctgagcctgagccacagccccggcaag

SEQ ID NO: 126 - protein, 216 aa, Canis lupus
  source 1..216: note = Canis familiaris
LGGPSVLIFPPKPKDILRITRTPEVTCVVLDLGREDPEVQISWFVDGKEVHTAKTQSREQQFNGTYRVVSVLPIEHQDWLTGKEFKCRVNHIDLPSPIERTISKARGRAHKPSVYVLPPSPKELSSSDTVSITCLIKDFYPPDIDVEWQSNGQQEPERKHRMTPPQLDEDGSYFLYSKLSVDKSRWQQGDPFTCAVMHETLQNHYTDLSLSHSPGK

SEQ ID NO: 127 - DNA, 648 bp, Canis lupus
  source 1..648: mol_type = unassigned DNA; note = Canis familiaris
ctgggcggccccagcgtgttcatcttcccccccaagcccaaggacatcctgagaatcaccagaacccccgagatcacctgcgtggtgctggacctgggcagagaggaccccgaggtgcagatcagctggttcgtggacggcaaggaggtgcacaccgccaagacccagcccagagagcagcagttcaacagcacctacagagtggtgagcgtgctgcccatcgagcaccaggactggctgaccggcaaggagttcaagtgcagagtgaaccacatcggcctgcccagccccatcgagagaaccatcagcaaggccagaggccaggcccaccagcccagcgtgtacgtgctgccccccagccccaaggagctgagcagcagcgacaccgtgaccctgacctgcctgatcaaggacttcttcccccccgagatcgacgtggagtggcagagcaacggccagcccgagcccgagagcaagtaccacaccaccgccccccagctggacgaggacggcagctacttcctgtacagcaagctgagcgtggacaagagcagatggcagcagggcgacaccttcacctgcgccgtgatgcacgaggccctgcagaaccactacaccgacctgagcctgagccacagccccggcaag

SEQ ID NO: 128 - protein, 216 aa, Canis lupus
  source 1..216: note = Canis familiaris
LGGPSVFIFPPKPKDILRITRTPEITCVVLDLGREDPEVQISWFVDGKEVHTAKTQPREQQFNSTYRVVSVLPIEHQDWLTGKEFKCRVNHIGLPSPIERTISKARGQAHQPSVYVLPPSPKELSSSDTVTLTCLIKDFFPPEIDVEWQSNGQPEPESKYHTTAPQLDEDGSYFLYSKLSVDKSRWQQGDTFTCAVMHEALQNHYTDLSLSHSPGK

SEQ ID NO: 129 - DNA, 645 bp, Canis lupus
  source 1..645: mol_type = unassigned DNA; note = Canis familiaris
ctgggcggccccagcgtgttcatcttcccccccaagcccaaggacaccctgctgatcgccagaacccccgaggtgacctgcgtggtggtggacctggaccccgaggaccccgaggtgcagatcagctggttcgtggacggcaagcagatgcagaccgccaagacccagcccagagaggagcagttcaacggcacctacagagtggtgagcgtgctgcccatcggccaccaggactggctgaagggcaagcagttcacctgcaaggtgaacaacaaggccctgcccagccccatcgagagaaccatcagcaaggccagaggccaggcccaccagcccagcgtgtacgtgctgccccccagcagagaggagctgagcaagaacaccgtgagcctgacctgcctgatcaaggacttcttcccccccgacatcgacgtggagtggcagagcaacggccagcaggagcccgagagcaagtacagaaccacccccccccagctggacgaggacggcagctacttcctgtacagcaagctgagcgtggacaagagcagatggcagagaggcgacaccttcatctgcgccgtgatgcacgaggccctgcacaaccactacacccaggagagcctgagccacagccccggcaag

SEQ ID NO: 130 - protein, 215 aa, Canis lupus
  source 1..215: note = Canis familiaris
LGGPSVFIFPPKPKDTLLIARTPEVTCVVVDLDPEDPEVQISWFVDGKQMQTAKTQPREEQFNGTYRVVSVLPIGHQDWLKGKQFTCKVNNKALPSPIERTISKARGQAHQPSVYVLPPSREELSKNTVSLTCLIKDFFPPDIDVEWQSNGQQEPESKYRTTPPQLDEDGSYFLYSKLSVDKSRWQRGDTFICAVMHEALHNHYTQESLSHSPGK

SEQ ID NO: 131 - DNA, 645 bp, Canis lupus
  source 1..645: mol_type = unassigned DNA; note = Canis familiaris
ctgggcggccccagcgtgttcatcttcccccccaagcccaaggacatcctggtgaccgccagaacccccaccgtgacctgcgtggtggtggacctggaccccgagaaccccgaggtgcagatcagctggttcgtggacagcaagcaggtgcagaccgccaacacccagcccagagaggagcagagcaacggcacctacagagtggtgagcgtgctgcccatcggccaccaggactggctgagcggcaagcagttcaagtgcaaggtgaacaacaaggccctgcccagccccatcgaggagatcatcagcaagacccccggccaggcccaccagcccaacgtgtacgtgctgccccccagcagagacgagatgagcaagaacaccgtgaccctgacctgcctggtgaaggacttcttcccccccgagatcgacgtggagtggcagagcaacggccagcaggagcccgagagcaagtacagaatgacccccccccagctggacgaggacggcagctacttcctgtacagcaagctgagcgtggacaagagcagatggcagagaggcgacaccttcatctgcgccgtgatgcacgaggccctgcacaaccactacacccagatcagcctgagccacagccccggcaag

SEQ ID NO: 132 - protein, 215 aa, Canis lupus
  source 1..215: note = Canis familiaris
LGGPSVFIFPPKPKDILVTARTPTVTCVVVDLDPENPEVQISWFVDSKQVQTANTQPREEQSNGTYRVVSVLPIGHQDWLSGKQFKCKVNNKALPSPIEEIISKTPGQAHQPNVYVLPPSRDEMSKNTVTLTCLVKDFFPPEIDVEWQSNGQQEPESKYRMTPPQLDEDGSYFLYSKLSVDKSRWQRGDTFICAVMHEALHNHYTQISLSHSPGK

SEQ ID NO: 133 - DNA, 867 bp, Canis lupus
  source 1..867: mol_type = unassigned DNA; note = Canis familiaris
atggggagccggcgggggccctggccgctcgtctgggccgtgctgcagctgggctggtggccaggatggctcctagactcccctgacaggccctggagcccgctcaccttctccccggcgcagctcacggtgcaggagggagagaacgccacgttcacctgcagcctggccgacatccccgacagcttcgtgctcaactggtaccgcctgagcccccgcaaccagacggacaagctggccgccttccaggaggaccgcatcgagccgggccgggacaggcgcttccgcgtcatgcggctgcccaacgggcgggacttccacatgagcatcgtcgctgcgcgcctcaacgacagcggcatctacctgtgcggggccatctacctgccccccaacacacagatcaacgagagtccccgcgcagagctctccgtgacggagagaaccctggagccccccacacagagccccagccccccacccagactcagcggccagttgcaggggctggtcatcggcgtcacgagcgtgctggtgggtgtcctgctactgctgctgctgacctgggtcctggccgctgtcttccccagggccacccgaggtgcctgtgtgtgcgggagcgaggacgagcctctgaaggagggccccgatgcagcgcccgtcttcaccctggactacggggagctggacttccagtggcgagagaagacgccggagcccccggcgccctgtgccccggagcagaccgagtatgccaccatcgtcttcccgggcaggccggcgtccccgggccgcagggcctcggccagcagcctgcagggagcccagcctccgagccccgaggacggacccggcctgtggcccctctga

SEQ ID NO: 134 - protein, 288 aa, Canis lupus
  source 1..288: note = Canis familiaris
MGSRRGPWPLVWAVLQLGWWPGWLLDSPDRPWSPLTFSPAQLTVQEGENATFTCSLADIPDSFVLNWYRLSPRNQTDKLAAFQEDRIEPGRDRRFRVMRLPNGRDFHMSIVAARLNDSGIYLCGAIYLPPNTQINESPRAELSVTERTLEPPTQSPSPPPRLSGQLQGLVIGVTSVLVGVLLLLLLTWVLAAVFPRATRGACVCGSEDEPLKEGPDAAPVFTLDYGELDFQWREKTPEPPAPCAPEQTEYATIVFPGRPASPGRRASASSLQGAQPPSPEDGPGLWPL

SEQ ID NO: 135 - DNA, 870 bp, Canis lupus
  source 1..870: mol_type = unassigned DNA; note = Canis familiaris
atgagaatgtttagtgtctttacattcatggcctactgccatttgctaaaagcatttacgatcacagtttctaaggacctgtatgtggtagagtatggtggcaatgtgacaatggaatgcaaattcccggtggaaaaacagttaaacttgtttgcactaatcgtctactgggaaatggaggataaaaaaattatacaatttgtgaatggaaaggaagacctgaaagttcagcacagcagctacagccagagggctcagctattgaaggaccagctcttcttggggaaggctgcgcttcagatcacagatgtgagattgcaggatgcaggggtttactgctgcttgatcggctatggcggtgctgactacaagcggattactttgaaagttcatgccccgtaccgcaacatcagccaaagaatttctgtggatcctgtcacctctgaacatgaactaatgtgtcaggctgagggttaccctgaggctgaagtcatctggacaagcagtgaccaccgagtcctgagtggcaaaaccaccatcactaattccaatagggaagagaagcttttcaatgtgaccagcacgctgaacatcaatgcaacagctaatgagattttctactgcacttttcaaagatcaggtcctgaggaaaacaatactgccgagttggtcatcccagaacgactgcccgttccagcaagtgagaggactcatttcatgattctgggacctttcctgttgcttcttggtgtagtcctggcagtcactttctgtctaaaaaaacatgggagaatgatggatgtggaaaaatgttgcacccgagataggaactcaaagaaacgaaatgatatacaatttgaagagacataa

SEQ ID NO: 136 - protein, 289 aa, Canis lupus
  source 1..289: note = Canis familiaris
MRMFSVFTFMAYCHLLKAFTITVSKDLYVVEYGGNVTMECKFPVEKQLNLFALIVYWEMEDKKIIQFVNGKEDLKVQHSSYSQRAQLLKDQLFLGKAALQITDVRLQDAGVYCCLIGYGGADYKRITLKVHAPYRNISQRISVDPVTSEHELMCQAEGYPEAEVIWTSSDHRVLSGKTTITNSNREEKLFNVTSTLNINATANEIFYCTFQRSGPEENNTAELVIPERLPVPASERTHFMILGPFLLLLGVVLAVTFCLKKHGRMMDVEKCCTRDRNSKKRNDIQFEET

SEQ ID NO: 137 - protein, 401 aa, Canis lupus
  source 1..401: note = Canis familiaris
MNFLLSWVHWSLALLLYLHHAKWSQALDSPDRPWSPLTFSPAQLTVQEGENATFTCSLADIPDSFVLNWYRLSPRNQTDKLAAFQEDRIEPGRDRRFRVMRLPNGRDFHMSIVAARLNDSGIYLCGAIYLPPNTQINESPRAELSVTERTLEPPTQSPSPPPRLSGQLQGLVGTDKTHTCPPCPAPELLGGPSVFLFPPKPKDTLMISRTPEVTCVVVDVSHEDPEVKFNWYVDGVEVHNAKTKPREEQYNSTYRVVSVLTVLHQDWLNGKEYKCKVSNKALPAPIEKTISKAKGQPREPQVYTLPPSRDELTKNQVSLTCLVKGFYPSDIAVEWESNGQPENNYKTTPPVLDSDGSFFLYSKLTVDKSRWQQGNVFSCSVMHEALHNHYTQKSLSLSPGK

SEQ ID NO: 138 - protein, 15 aa, Canis lupus
  VARIANT 9: note = misc_feature - Xaa can be Met or Thr
  source 1..15: note = Canis familiaris
GRDRRFRVXRLPNGR

SEQ ID NO: 139 - protein, 15 aa, Canis lupus
  VARIANT 14: note = MISC_FEATURE - Xaa can be Met or Thr
  source 1..15: note = Canis familiaris
DRIEPGRDRRFRVXR

SEQ ID NO: 140 - protein, 25 aa, Canis lupus
  VARIANT 5: note = MISC_FEATURE - Xaa can be Met or Thr
  source 1..25: note = Canis familiaris
RFRVXRLPNGRDFHMSIVAARLNDS

SEQ ID NO: 141 - protein, 26 aa, Canis lupus
  VARIANT 20: note = MISC_FEATURE - Xaa can be Met or Thr
  source 1..26: note = Canis familiaris
LAAFQEDRIEPGRDRRFRVXRLPNGR

SEQ ID NO: 142 - protein, 31 aa, Canis lupus
  VARIANT 15: note = MISC_FEATURE - Xaa can be Met or Thr
  source 1..31: note = Canis familiaris
EDRIEPGRDRRFRVXRLPNGRDFHMSIVAAR

SEQ ID NO: 143 - protein, 31 aa, Canis lupus
  VARIANT 25: note = MISC_FEATURE - Xaa can be Met or Thr
  source 1..31: note = Canis familiaris
NQTDKLAAFQEDRIEPGRDRRFRVXRLPNGR

SEQ ID NO: 144 - protein, 45 aa, Canis lupus
  VARIANT 25: note = MISC_FEATURE - Xaa can be Met or Thr
  source 1..45: note = Canis familiaris
NQTDKLAAFQEDRIEPGRDRRFRVXRLPNGRDFHMSIVAARLNDS

SEQ ID NO: 145 - protein, 20 aa, Canis lupus
  VARIANT 14: note = MISC_FEATURE - Xaa can be Met or Thr
  source 1..20: note = Canis familiaris
DRIEPGRDRRFRVXRLPNGR

SEQ ID NO: 146 - protein, 11 aa, Mus musculus
IFYDYDGDIDV